European Patent Application EP 4 353 737 A1, published April 17, 2024. Title: Fusion proteins comprising a cell surface marker specific VHH. Applicant: UNIVERSITÄTSKLINIKUM HAMBURG-EPPENDORF. Application EP. The sequence listing filed with the application follows.

SEQUENCE LISTING (65 sequences)

SEQ ID NO: 1 - protein, 879 aa, synthetic construct
MAADGYLPDWLEDNLSEGIREWWALKPGAPQPKANQQHQDNARGLVLPGYKYLGPGNGLDKGEPVNAADAAALEHDKAYDQQLKAGDNPYLKYNHADAEFQERLKEDTSFGGNLGRAVFQAKKRLLEPLGLVEEAAKTAPGKKRPVEQSPQEPDSSAGIGKSGAQPAKKRLNFGQTGDTESVPDPQPIGEPPAAPSGVGSLTMASGGGAPVADNNEGADGVGSSSGNWHCDSQWLGDRVITTSTRTWALPTYNNHLYKQISNSTSGGSSNDNAYFGYSTPWGYFDFNRFHCHFSPRDWQRLINNNWGFRPKRLNFKLFNIQVKEVTDNNGVKTIANNLTSTVQVFTDSDYQLPYVLGSAHEGCLPPFPADVFMIPQYGYLTLNDGSQAVGRSSFYCLEYFPSQMLRTGNNFQFSYEFENVPFHSSYAHSQSLDRLMNPLIDQYLYYLSKTIDGAGGGGSGGGGSGGGGSGGGGSGGDMSQVQLVESGGGRVQTGGSLRLSCAASGISFSITTMYWYRQAPGEQRQLVALITDRGNTYYVDSVKGRFTISRDDSKNTVYLQMNDLKPEDTAVYFCNSIPGNDWGQGTQVTVSSAAAGAGQNQQTLKFSVAGPSNMAVQGRNYIPGPSYRQQRVSTTVTQNNNSEFAAPGASSWALNGRNSLMNPGPAMASHKEGEDRFFPLSGSLIFGKQGTGRDNVDADKVMITNEEEIKTTNPVATESYGQVATNHQSAQAQAQTGWVQNQGILPGMVWQDRDVYLQGPIWAKIPHTDGNFHPSPLMGGFGMKHPPPQILIKNTPVPADPPTAFNKDKLNSFITQYSTGQVSVEIEWELQKENSKRWNPEIQYTSNYYKSNNVEFAVNTEGVYSEPRPIGTRYLTRNL

SEQ ID NO: 2 - DNA, 2641 bp, synthetic construct
  source 1..2641: mol_type = other DNA
atggccgctgatggctatctacccgattggcttgaggacaacctgtccgaaggaatcagggagtggtgggcgttgaaaccaggagccccgcaaccgaaggccaatcaacaacatcaagacaacgcccggggacttgtcctgccaggctacaaatacttgggacccggcaacggactggacaagggcgagccagtaaacgcggctgacgcggcggctctggagcacgacaaggcctacgaccagcagttgaaggccggtgacaacccgtacctcaagtacaaccacgccgacgccgagttccaggagcggcttaaggaagatactagttttggcggaaacctcggtagggctgttttccaggccaagaagcggctgcttgaacccttgggcctggttgaggaagctgctaaaaccgccccaggaaagaaacgtccagtggagcagagtccccaggaaccagactcctcagctggtattggcaaaagtggcgcacaaccggctaagaagcgactcaatttcggccagaccggggatactgagtccgttcctgatccgcaacctattggagagccgcccgcggccccaagcggcgtgggctctttgactatggcttccggtggcggcgctcctgtggccgacaacaacgaaggagctgatggagtgggatcatcctcaggtaattggcattgcgatagccaatggcttggggacagagtgatcacaacatccacccgcacgtgggccttgccaacatacaacaatcacctgtacaagcaaatcagtaactcaaccagcggtggaagcagtaatgacaacgcgtacttcggttactctaccccttggggatattttgacttcaaccgtttccactgccacttctcaccgagagactggcagcgcctcataaataacaactggggattccgccccaagcgactgaacttcaagttgttcaacatccaggttaaagaggtgactgacaacaatggtgtgaagacaatcgccaataacctcacgagtaccgtccaggtcttcactgacagtgattatcaactgccctacgtgcttggatctgctcacgagggatgcctgcccccattccccgctgacgttttcatgattcctcagtacggctatctgacactcaatgatggcagccaggcggtcggtaggtcctcattttactgcctcgaatatttcccttcacaaatgctgcgcacggggaacaacttccagttctcctacgagtttgagaacgtcccattccatagcagctacgctcactctcaatctctggacaggctcatgaatcctctcatcgaccaatacctgtactatttgagcaagacaattgacggtgccggcggcggcgggagtggcggaggaggatcaggcggaggagggagtggtggaggaggttcaggcggggacatgtcacaagttcagttggtggagtctggcggtggacgagtgcagacgggcgggtccctgagactgtcctgtgcagcatcaggcatcagcttcagtatcaccaccatgtactggtaccgccaggccccaggagagcagaggcagctggtcgctttgattactgatcggggaaacacctactatgttgactcagtgaagggacgcttcaccatcagtcgtgacgactctaagaacacagtctatctccaaatgaacgacctgaaacctgaggacacagctgtgtatttctgtaattccatccctgggaacgactggggccagggtactcaggtcacagtcagttccgcggccgctggcgccgggcaaaatcagcagacactcaaattctcagttgcagggccttctaacatggccgttcagggccgtaactacattccgggcccctcataccgacaacaacgcgtgagtactactgttacacaaaacaacaactccgaatttgctgcgctggccaggagcctcaagctgggctcttaatggtcgtaattccctgatgaatcctgggcccgcgatggccagtcacaaagagggcgaggaccgattctttccactcagcggaagcttgatctttggaaaacaagggacgggtcgcgacaacgttgatgccgacaaagttatgataaccaacgaggaagaaatcaaaacaacgaacccggttgctactgagtcttatggtcaagttgccaccaaccaccagtccgcccaagcacaggctcagaccggttgggtgcaaaaccaaggcatcttgcctggcatggtttggcaggaccgcgatgtttatctccaaggacccatttgggccaaaattcctcacacggacgggaactttcacccatcacctctgatgggcggctttggcatgaagcatcccccaccccagatcctcatcaagaacacgcctgtacccgcagatcccccgaccgccttcaacaaggacaagctgaactccttcatcacacagtattccacagggcaagtctcagttgagatcgagtgggagctgcaaaaggaaaacagcaagcgctggaaccccgagatccagtacacgtcaaactattacaagtctaataatgtcgaatttgccgtgaatacggaaggtgtgtattccgaacctcggcccataggcactcggtacctgactagaaatttg

SEQ ID NO: 3 - protein, 881 aa, synthetic construct
MAADGYLPDWLEDNLSEGIREWWALKPGAPQPKANQQHQDNARGLVLPGYKYLGPGNGLDKGEPVNAADAAALEHDKAYDQQLKAGDNPYLKYNHADAEFQERLKEDTSFGGNLGRAVFQAKKRLLEPLGLVEEAAKTAPGKKRPVEQSPQEPDSSAGIGKSGAQPAKKRLNFGQTGDTESVPDPQPIGEPPAAPSGVGSLTMASGGGAPVADNNEGADGVGSSSGNWHCDSQWLGDRVITTSTRTWALPTYNNHLYKQISNSTSGGSSNDNAYFGYSTPWGYFDFNRFHCHFSPRDWQRLINNNWGFRPKRLNFKLFNIQVKEVTDNNGVKTIANNLTSTVQVFTDSDYQLPYVLGSAHEGCLPPFPADVFMIPQYGYLTLNDGSQAVGRSSFYCLEYFPSQMLRTGNNFQFSYEFENVPFHSSYAHSQSLDRLMNPLIDQYLYYLSKTIDGAGGGGSGGGGSGGGGSGGGGSGGDMSDVQLQASGGGSVQAGGSLTLSCRYSGGFVFRVSSMGWYRQAPGNQRELIATITVGGKTNYKDSVQRFIISRNDTTVTLQMNRLQPEDTAVYYCNLASTAVGADTWGQGTRVTVSSAAAGAGQNQQTLKFSVAGPSNMAVQGRNYIPGPSYRQQRVSTTVTQNNNSEFAAPGASSWALNGRNSLMNPGPAMASHKEGEDRFFPLSGSLIFGKQGTGRDNVDADKVMITNEEEIKTTNPVATESYGQVATNHQSAQAQAQTGWVQNQGILPGMVWQDRDVYLQGPIWAKIPHTDGNFHPSPLMGGFGMKHPPPQILIKNTPVPADPPTAFNKDKLNSFITQYSTGQVSVEIEWELQKENSKRWNPEIQYTSNYYKSNNVEFAVNTEGVYSEPRPIGTRYLTRNL

SEQ ID NO: 4 - DNA, 2640 bp, synthetic construct
  source 1..2640: mol_type = other DNA
atggccgctgatggctatctacccgattggcttgaggacaacctgtccgaaggaatcagggagtggtgggcgttgaaaccaggagccccgcaaccgaaggccaatcaacaacatcaagacaacgcccggggacttgtcctgccaggctacaaatacttgggacccggcaacggactggacaagggcgagccagtaaacgcggctgacgcggcggctctggagcacgacaaggcctacgaccagcagttgaaggccggtgacaacccgtacctcaagtacaaccacgccgacgccgagttccaggagcggcttaaggaagatactagttttggcggaaacctcggtagggctgttttccaggccaagaagcggctgcttgaacccttgggcctggttgaggaagctgctaaaaccgccccaggaaagaaacgtccagtggagcagagtccccaggaaccagactcctcagctggtattggcaaaagtggcgcacaaccggctaagaagcgactcaatttcggccagaccggggatactgagtccgttcctgatccgcaacctattggagagccgcccgcggccccaagcggcgtgggctctttgactatggcttccggtggcggcgctcctgtggccgacaacaacgaaggagctgatggagtgggatcatcctcaggtaattggcattgcgatagccaatggcttggggacagagtgatcacaacatccacccgcacgtgggccttgccaacatacaacaatcacctgtacaagcaaatcagtaactcaaccagcggtggaagcagtaatgacaacgcgtacttcggttactctaccccttggggatattttgacttcaaccgtttccactgccacttctcaccgagagactggcagcgcctcataaataacaactggggattccgccccaagcgactgaacttcaagttgttcaacatccaggttaaagaggtgactgacaacaatggtgtgaagacaatcgccaataacctcacgagtaccgtccaggtcttcactgacagtgattatcaactgccctacgtgcttggatctgctcacgagggatgcctgcccccattccccgctgacgttttcatgattcctcagtacggctatctgacactcaatgatggcagccaggcggtcggtaggtcctcattttactgcctcgaatatttcccttcacaaatgctgcgcacggggaacaacttccagttctcctacgagtttgagaacgtcccattccatagcagctacgctcactctcaatctctggacaggctcatgaatcctctcatcgaccaatacctgtactatttgagcaagacaattgacggtgccggcggcggcgggagtggcggaggaggatcaggcggaggagggagtggtggaggaggttcaggcggggatgtgcagctgcaggcgtctgggggaggctcggtgcaggctggagggtctctgacgctctcctgtagatactctggtggattcgtctttagagtcagtagtatgggctggtaccgccaggctccagggaaccagcgcgagttgatcgcaacgattactgttggcgggaaaacaaactataaagactccgtacagggccgatttatcatctccagaaacgatacgacggtgacgctacagatgaatagactgcaacctgaggacacagccgtctattactgtaatttagcatcaacggcagttggagccgacacctggggccaggggacccgggtcaccgtctcctcagcggccgctggcgccgggcaaaatcagcagacactcaaattctcagttgcagggccttctaacatggccgttcagggccgtaactacattccgggcccctcataccgacaacaacgcgtgagtactactgttacacaaaacaacaactccgaatttgcttggccaggagcctcaagctgggctcttaatggtcgtaattccctgatgaatcctgggcccgcgatggccagtcacaaagagggcgaggaccgattctttccactcagcggaagcttgatctttggaaaacaagggacgggtcgcgacaacgttgatgccgacaaagttatgataaccaacgaggaagaaatcaaaacaacgaacccggttgctactgagtcttatggtcaagttgccaccaaccaccagtccgcccaagcacaggctcagaccggttgggtgcaaaaccaaggcatcttgcctggcatggtttggcaggaccgcgatgtttatctccaaggacccatttgggccaaaattcctcacacggacgggaactttcacccatcacctctgatgggcggctttggcatgaagcatcccccaccccagatcctcatcaagaacacgcctgtacccgcagatcccccgaccgccttcaacaaggacaagctgaactccttcatcacacagtattccacagggcaagtctcagttgagatcgagtgggagctgcaaaaggaaaacagcaagcgctggaaccccgagatccagtacacgtcaaactattacaagtctaataatgtcgaatttgccgtgaatacggaaggtgtgtattccgaacctcggcccataggcactcggtacctgactagaaatttgtga

SEQ ID NO: 5 - protein, 890 aa, synthetic construct
MAADGYLPDWLEDNLSEGIREWWALKPGAPQPKANQQHQDNARGLVLPGYKYLGPGNGLDKGEPVNAADAAALEHDKAYDQQLKAGDNPYLKYNHADAEFQERLKEDTSFGGNLGRAVFQAKKRLLEPLGLVEEAAKTAPGKKRPVEQSPQEPDSSAGIGKSGAQPAKKRLNFGQTGDTESVPDPQPIGEPPAAPSGVGSLTMASGGGAPVADNNEGADGVGSSSGNWHCDSQWLGDRVITTSTRTWALPTYNNHLYKQISNSTSGGSSNDNAYFGYSTPWGYFDFNRFHCHFSPRDWQRLINNNWGFRPKRLNFKLFNIQVKEVTDNNGVKTIANNLTSTVQVFTDSDYQLPYVLGSAHEGCLPPFPADVFMIPQYGYLTLNDGSQAVGRSSFYCLEYFPSQMLRTGNNFQFSYEFENVPFHSSYAHSQSLDRLMNPLIDQYLYYLSKTIDGAGGGGSGGGGSGGGGSGGGGSGGDMSDVQLQESGGGLVQAGGSLRLSCTGSGRTFRNYPMAWFRQAPGKEREFVAGITWVGASTLYADFAKGRFTISRDNAKNTVYLQMNSLKPEDTAVYSCAAGRGIVAGRIPAEYADWGQGTQVTVSSAAAGAGQNQQTLKFSVAGPSNMAVQGRNYIPGPSYRQQRVSTTVTQNNNSEFAAPGASSWALNGRNSLMNPGPAMASHKEGEDRFFPLSGSLIFGKQGTGRDNVDADKVMITNEEEIKTTNPVATESYGQVATNHQSAQAQAQTGWVQNQGILPGMVWQDRDVYLQGPIWAKIPHTDGNFHPSPLMGGFGMKHPPPQILIKNTPVPADPPTAFNKDKLNSFITQYSTGQVSVEIEWELQKENSKRWNPEIQYTSNYYKSNNVEFAVNTEGVYSEPRPIGTRYLTRNL

SEQ ID NO: 6 - DNA, 2583 bp, synthetic construct
  source 1..2583: mol_type = other DNA
atggccgctgatggctatctacccgattggcttgaggacaacctgtccgaaggaatcagggagtggtgggcgttgaaaccaggagccccgcaaccgaaggccaatcaacaacatcaagacaacgcccggggacttgtcctgccaggctacaaatacttgggacccggcaacggactggacaagggcgagccagtaaacgcggctgacgcggcggctctggagcacgacaaggcctacgaccagcagttgaaggccggtgacaacccgtacctcaagtacaaccacgccgacgccgagttccaggagcggcttaaggaagatactagttttggcggaaacctcggtagggctgttttccaggccaagaagcggctgcttgaacccttgggcctggttgaggaagctgctaaaaccgccccaggaaagaaacgtccagtggagcagagtccccaggaaccagactcctcagctggtattggcaaaagtggcgcacaaccggctaagaagcgactcaatttcggccagaccggggatactgagtccgttcctgatccgcaacctattggagagccgcccgcggccccaagcggcgtgggctctttgactatggcttccggtggcggcgctcctgtggccgacaacaacgaaggagctgatggagtgggatcatcctcaggtaattggcattgcgatagccaatggcttggggacagagtgatcacaacatccacccgcacgtgggccttgccaacatacaacaatcacctgtacaagcaaatcagtaactcaaccagcggtggaagcagtaatgacaacgcgtacttcggttactctaccccttggggatattttgacttcaaccgtttccactgccacttctcaccgagagactggcagcgcctcataaataacaactggggattccgccccaagcgactgaacttcaagttgttcaacatccaggttaaagaggtgactgacaacaatggtgtgaagacaatcgccaataacctcacgagtaccgtccaggtcttcactgacagtgattatcaactgccctacgtgcttggatctgctcacgagggatgcctgcccccattccccgctgacgttttcatgattcctcagtacggctatctgacactcaatgatggcagccaggcggtcggtaggtcctcattttactgcctcgaatatttcccttcacaaatgctgcgcacggggaacaacttccagttctcctacgagtttgagaacgtcccattccatagcagctacgctcactctcaatctctggacaggctcatgaatcctctcatcgaccaatacctgtactatttgagcaagacaattgacggtgccgatgtgcagctgcaggagtctggaggaggcttggtgcaggctgggggctctctgagactctcctgtacaggctcaggacgcaccttcaggaactatcccatggcctggttccgccaggctccaggaaaggagcgtgagtttgtagcaggtattacctgggtcggtgctagcacactctatgcagacttcgcgaagggccgattcaccatctccagagacaacgccaagaacacggtgtatctgcaaatgaacagcctgaaacctgaggacacggccgtttatagttgtgcagcaggtcgcggtatagtggctggtaggatcccagctgagtatgccgactggggccagggcacccaggtcaccgtctcctcagggcaaaatcagcagacactcaaattctcagttgcagggccttctaacatggccgttcagggccgtaactacattccgggcccctcataccgacaacaacgcgtgagtactactgttacacaaaacaacaactccgaatttgcttggccaggagcctcaagctgggctcttaatggtcgtaattccctgatgaatcctgggcccgcgatggccagtcacaaagagggcgaggaccgattctttccactcagcggaagcttgatctttggaaaacaagggacgggtcgcgacaacgttgatgccgacaaagttatgataaccaacgaggaagaaatcaaaacaacgaacccggttgctactgagtcttatggtcaagttgccaccaaccaccagtccgcccaagcacaggctcagaccggttgggtgcaaaaccaaggcatcttgcctggcatggtttggcaggaccgcgatgtttatctccaaggacccatttgggccaaaattcctcacacggacgggaactttcacccatcacctctgatgggcggctttggcatgaagcatcccccaccccagatcctcatcaagaacacgcctgtacccgcagatcccccgaccgccttcaacaaggacaagctgaactccttcatcacacagtattccacagggcaagtctcagttgagatcgagtgggagctgcaaaaggaaaacagcaagcgctggaaccccgagatccagtacacgtcaaactattacaagtctaataatgtcgaatttgccgtgaatacggaaggtgtgtattccgaacctcggcccataggcactcggtacctgactagaaatttgtga

SEQ ID NO: 7 - protein, 894 aa, synthetic construct
MAADGYLPDWLEDNLSEGIREWWALKPGAPQPKANQQHQDNARGLVLPGYKYLGPGNGLDKGEPVNAADAAALEHDKAYDQQLKAGDNPYLKYNHADAEFQERLKEDTSFGGNLGRAVFQAKKRLLEPLGLVEEAAKTAPGKKRPVEQSPQEPDSSAGIGKSGAQPAKKRLNFGQTGDTESVPDPQPIGEPPAAPSGVGSLTMASGGGAPVADNNEGADGVGSSSGNWHCDSQWLGDRVITTSTRTWALPTYNNHLYKQISNSTSGGSSNDNAYFGYSTPWGYFDFNRFHCHFSPRDWQRLINNNWGFRPKRLNFKLFNIQVKEVTDNNGVKTIANNLTSTVQVFTDSDYQLPYVLGSAHEGCLPPFPADVFMIPQYGYLTLNDGSQAVGRSSFYCLEYFPSQMLRTGNNFQFSYEFENVPFHSSYAHSQSLDRLMNPLIDQYLYYLSKTIDGAGGGGSGGGGSGGGGSGGGGSGGDMSDVQLQESGGGLVQAGDSLRLSCVGSGRRFDNYAMAWFRQAPGKERTFVAAISWSSGTTRYLDTVKGRFTISRDNAKSTVYLQMNSLKPEDTAVYYCAARYQPRYYDSGDMDGYEYEFWGQGTQVTVSSAAAGAGQNQQTLKFSVAGPSNMAVQGRNYIPGPSYRQQRVSTTVTQNNNSEFAAPGASSWALNGRNSLMNPGPAMASHKEGEDRFFPLSGSLIFGKQGTGRDNVDADKVMITNEEEIKTTNPVATESYGQVATNHQSAQAQAQTGWVQNQGILPGMVWQDRDVYLQGPIWAKIPHTDGNFHPSPLMGGFGMKHPPPQILIKNTPVPADPPTAFNKDKLNSFITQYSTGQVSVEIEWELQKENSKRWNPEIQYTSNYYKSNNVEFAVNTEGVYSEPRPIGTRYLTRNL

SEQ ID NO: 8 - DNA, 2595 bp, synthetic construct
  source 1..2595: mol_type = other DNA
atggccgctgatggctatctacccgattggcttgaggacaacctgtccgaaggaatcagggagtggtgggcgttgaaaccaggagccccgcaaccgaaggccaatcaacaacatcaagacaacgcccggggacttgtcctgccaggctacaaatacttgggacccggcaacggactggacaagggcgagccagtaaacgcggctgacgcggcggctctggagcacgacaaggcctacgaccagcagttgaaggccggtgacaacccgtacctcaagtacaaccacgccgacgccgagttccaggagcggcttaaggaagatactagttttggcggaaacctcggtagggctgttttccaggccaagaagcggctgcttgaacccttgggcctggttgaggaagctgctaaaaccgccccaggaaagaaacgtccagtggagcagagtccccaggaaccagactcctcagctggtattggcaaaagtggcgcacaaccggctaagaagcgactcaatttcggccagaccggggatactgagtccgttcctgatccgcaacctattggagagccgcccgcggccccaagcggcgtgggctctttgactatggcttccggtggcggcgctcctgtggccgacaacaacgaaggagctgatggagtgggatcatcctcaggtaattggcattgcgatagccaatggcttggggacagagtgatcacaacatccacccgcacgtgggccttgccaacatacaacaatcacctgtacaagcaaatcagtaactcaaccagcggtggaagcagtaatgacaacgcgtacttcggttactctaccccttggggatattttgacttcaaccgtttccactgccacttctcaccgagagactggcagcgcctcataaataacaactggggattccgccccaagcgactgaacttcaagttgttcaacatccaggttaaagaggtgactgacaacaatggtgtgaagacaatcgccaataacctcacgagtaccgtccaggtcttcactgacagtgattatcaactgccctacgtgcttggatctgctcacgagggatgcctgcccccattccccgctgacgttttcatgattcctcagtacggctatctgacactcaatgatggcagccaggcggtcggtaggtcctcattttactgcctcgaatatttcccttcacaaatgctgcgcacggggaacaacttccagttctcctacgagtttgagaacgtcccattccatagcagctacgctcactctcaatctctggacaggctcatgaatcctctcatcgaccaatacctgtactatttgagcaagacaattgacggtgccgatgtgcagctgcaggagtctggaggaggattggtgcaggctggggactctctgagactctcctgtgtaggctctggacgcaggttcgataattatgccatggcgtggttccgccaggctccaggaaaggagcgtacatttgtagcagctattagctggagtagtggcactacgcgctatttagataccgtgaagggccgattcaccatatccagagacaacgccaagtctacggtgtatcttcaaatgaacagcctgaaacctgaggacacggccgtttattactgtgcagctcgataccagccgaggtactacgactcaggggatatggatggatatgagtatgaattctggggtcaggggacccaggtcaccgtctcctcagggcaaaatcagcagacactcaaattctcagttgcagggccttctaacatggccgttcagggccgtaactacattccgggcccctcataccgacaacaacgcgtgagtactactgttacacaaaacaacaactccgaatttgcttggccaggagcctcaagctgggctcttaatggtcgtaattccctgatgaatcctgggcccgcgatggccagtcacaaagagggcgaggaccgattctttccactcagcggaagcttgatctttggaaaacaagggacgggtcgcgacaacgttgatgccgacaaagttatgataaccaacgaggaagaaatcaaaacaacgaacccggttgctactgagtcttatggtcaagttgccaccaaccaccagtccgcccaagcacaggctcagaccggttgggtgcaaaaccaaggcatcttgcctggcatggtttggcaggaccgcgatgtttatctccaaggacccatttgggccaaaattcctcacacggacgggaactttcacccatcacctctgatgggcggctttggcatgaagcatcccccaccccagatcctcatcaagaacacgcctgtacccgcagatcccccgaccgccttcaacaaggacaagctgaactccttcatcacacagtattccacagggcaagtctcagttgagatcgagtgggagctgcaaaaggaaaacagcaagcgctggaaccccgagatccagtacacgtcaaactattacaagtctaataatgtcgaatttgccgtgaatacggaaggtgtgtattccgaacctcggcccataggcactcggtacctgactagaaatttgtga

SEQ ID NO: 9 - protein, 878 aa, synthetic construct
MAADGYLPDWLEDNLSEGIREWWALKPGAPQPKANQQHQDNARGLVLPGYKYLGPGNGLDKGEPVNAADAAALEHDKAYDQQLKAGDNPYLKYNHADAEFQERLKEDTSFGGNLGRAVFQAKKRLLEPLGLVEEAAKTAPGKKRPVEQSPQEPDSSAGIGKSGAQPAKKRLNFGQTGDTESVPDPQPIGEPPAAPSGVGSLTMASGGGAPVADNNEGADGVGSSSGNWHCDSQWLGDRVITTSTRTWALPTYNNHLYKQISNSTSGGSSNDNAYFGYSTPWGYFDFNRFHCHFSPRDWQRLINNNWGFRPKRLNFKLFNIQVKEVTDNNGVKTIANNLTSTVQVFTDSDYQLPYVLGSAHEGCLPPFPADVFMIPQYGYLTLNDGSQAVGRSSFYCLEYFPSQMLRTGNNFQFSYEFENVPFHSSYAHSQSLDRLMNPLIDQYLYYLSKTIDGAGGGGSGGGGSGGGGSGGGGSGGDQVQLVETGGGLVQPGGSLRLSCTASGFTFSMHAMTWYRQAPGKQRELVAVITSHGDRANYTDSVRGRFTISRDNTKNMVYLQMNSLKPEDTAVYYCNVPRYDSWGQGTQVTVSSAAAGAGQNQQTLKFSVAGPSNMAVQGRNYIPGPSYRQQRVSTTVTQNNNSEFAAPGASSWALNGRNSLMNPGPAMASHKEGEDRFFPLSGSLIFGKQGTGRDNVDADKVMITNEEEIKTTNPVATESYGQVATNHQSAQAQAQTGWVQNQGILPGMVWQDRDVYLQGPIWAKIPHTDGNFHPSPLMGGFGMKHPPPQILIKNTPVPADPPTAFNKDKLNSFITQYSTGQVSVEIEWELQKENSKRWNPEIQYTSNYYKSNNVEFAVNTEGVYSEPRPIGTRYLTRNL

SEQ ID NO: 10 - DNA, 2553 bp, synthetic construct
  source 1..2553: mol_type = other DNA
atggccgctgatggctatctacccgattggcttgaggacaacctgtccgaaggaatcagggagtggtgggcgttgaaaccaggagccccgcaaccgaaggccaatcaacaacatcaagacaacgcccggggacttgtcctgccaggctacaaatacttgggacccggcaacggactggacaagggcgagccagtaaacgcggctgacgcggcggctctggagcacgacaaggcctacgaccagcagttgaaggccggtgacaacccgtacctcaagtacaaccacgccgacgccgagttccaggagcggcttaaggaagatactagttttggcggaaacctcggtagggctgttttccaggccaagaagcggctgcttgaacccttgggcctggttgaggaagctgctaaaaccgccccaggaaagaaacgtccagtggagcagagtccccaggaaccagactcctcagctggtattggcaaaagtggcgcacaaccggctaagaagcgactcaatttcggccagaccggggatactgagtccgttcctgatccgcaacctattggagagccgcccgcggccccaagcggcgtgggctctttgactatggcttccggtggcggcgctcctgtggccgacaacaacgaaggagctgatggagtgggatcatcctcaggtaattggcattgcgatagccaatggcttggggacagagtgatcacaacatccacccgcacgtgggccttgccaacatacaacaatcacctgtacaagcaaatcagtaactcaaccagcggtggaagcagtaatgacaacgcgtacttcggttactctaccccttggggatattttgacttcaaccgtttccactgccacttctcaccgagagactggcagcgcctcataaataacaactggggattccgccccaagcgactgaacttcaagttgttcaacatccaggttaaagaggtgactgacaacaatggtgtgaagacaatcgccaataacctcacgagtaccgtccaggtcttcactgacagtgattatcaactgccctacgtgcttggatctgctcacgagggatgcctgcccccattccccgctgacgttttcatgattcctcagtacggctatctgacactcaatgatggcagccaggcggtcggtaggtcctcattttactgcctcgaatatttcccttcacaaatgctgcgcacggggaacaacttccagttctcctacgagtttgagaacgtcccattccatagcagctacgctcactctcaatctctggacaggctcatgaatcctctcatcgaccaatacctgtactatttgagcaagacaattgacggtgcccaagtacaattggtggagacaggtggtggtctggtgcaacccggcggtagcctgaggttgagttgcacagcttccggctttaccttcagcatgcatgcaatgacttggtatagacaggccccaggaaaacaacgggagctggtcgccgtgatcacatcacacggtgaccgggccaattacacagattctgtcaggggacggttcaccatttcacgtgataatacaaagaatatggtttatctccaaatgaatagccttaaaccagaggataccgctgtgtattactgtaatgtcccacgatatgattcctggggccagggaacacaagtaaccgttagcagcgggcaaaatcagcagacactcaaattctcagttgcagggccttctaacatggccgttcagggccgtaactacattccgggcccctcataccgacaacaacgcgtgagtactactgttacacaaaacaacaactccgaatttgcttggccaggagcctcaagctgggctcttaatggtcgtaattccctgatgaatcctgggcccgcgatggccagtcacaaagagggcgaggaccgattctttccactcagcggaagcttgatctttggaaaacaagggacgggtcgcgacaacgttgatgccgacaaagttatgataaccaacgaggaagaaatcaaaacaacgaacccggttgctactgagtcttatggtcaagttgccaccaaccaccagtccgcccaagcacaggctcagaccggttgggtgcaaaaccaaggcatcttgcctggcatggtttggcaggaccgcgatgtttatctccaaggacccatttgggccaaaattcctcacacggacgggaactttcacccatcacctctgatgggcggctttggcatgaagcatcccccaccccagatcctcatcaagaacacgcctgtacccgcagatcccccgaccgccttcaacaaggacaagctgaactccttcatcacacagtattccacagggcaagtctcagttgagatcgagtgggagctgcaaaaggaaaacagcaagcgctggaaccccgagatccagtacacgtcaaactattacaagtctaataatgtcgaatttgccgtgaatacggaaggtgtgtattccgaacctcggcccataggcactcggtacctgactagaaatttgtga

SEQ ID NO: 11 - protein, 879 aa, synthetic construct
MAADGYLPDWLEDNLSEGIREWWALKPGAPQPKANQQHQDNARGLVLPGYKYLGPGNGLDKGEPVNAADAAALEHDKAYDQQLKAGDNPYLKYNHADAEFQERLKEDTSFGGNLGRAVFQAKKRLLEPLGLVEEAAKTAPGKKRPVEQSPQEPDSSAGIGKSGAQPAKKRLNFGQTGDTESVPDPQPIGEPPAAPSGVGSLTMASGGGAPVADNNEGADGVGSSSGNWHCDSQWLGDRVITTSTRTWALPTYNNHLYKQISNSTSGGSSNDNAYFGYSTPWGYFDFNRFHCHFSPRDWQRLINNNWGFRPKRLNFKLFNIQVKEVTDNNGVKTIANNLTSTVQVFTDSDYQLPYVLGSAHEGCLPPFPADVFMIPQYGYLTLNDGSQAVGRSSFYCLEYFPSQMLRTGNNFQFSYEFENVPFHSSYAHSQSLDRLMNPLIDQYLYYLSKTIDGSGQNQQTLKFSVAGPSNMAVQGRNYIPGPSYRQQRVSTTVTQNNNSEFAAPGASSWALNGRNSLMNPGPAMASHKEGEDRFFPLSGSLIFGKQGTGRDNVDADKVMITNEEEIKTTNPVATESYGQVATNHQSAGGGGSGGGGSGGGGSGGGGSGGDMSQVQLVESGGGRVQTGGSLRLSCAASGISFSITTMYWYRQAPGEQRQLVALITDRGNTYYVDSVKGRFTISRDDSKNTVYLQMNDLKPEDTAVYFCNSIPGNDWGQGTQVTVSSAAAGAQAQAQTGWVQNQGILPGMVWQDRDVYLQGPIWAKIPHTDGNFHPSPLMGGFGMKHPPPQILIKNTPVPADPPTAFNKDKLNSFITQYSTGQVSVEIEWELQKENSKRWNPEIQYTSNYYKSNNVEFAVNTEGVYSEPRPIGTRYLTRNL

SEQ ID NO: 12 - DNA, 2637 bp, synthetic construct
  source 1..2637: mol_type = other DNA
atggccgctgatggctatctacccgattggcttgaggacaacctgtccgaaggaatcagggagtggtgggcgttgaaaccaggagccccgcaaccgaaggccaatcaacaacatcaagacaacgcccggggacttgtcctgccaggctacaaatacttgggacccggcaacggactggacaagggcgagccagtaaacgcggctgacgcggcggctctggagcacgacaaggcctacgaccagcagttgaaggccggtgacaacccgtacctcaagtacaaccacgccgacgccgagttccaggagcggcttaaggaagatactagttttggcggaaacctcggtagggctgttttccaggccaagaagcggctgcttgaacccttgggcctggttgaggaagctgctaaaaccgccccaggaaagaaacgtccagtggagcagagtccccaggaaccagactcctcagctggtattggcaaaagtggcgcacaaccggctaagaagcgactcaatttcggccagaccggggatactgagtccgttcctgatccgcaacctattggagagccgcccgcggccccaagcggcgtgggctctttgactatggcttccggtggcggcgctcctgtggccgacaacaacgaaggagctgatggagtgggatcatcctcaggtaattggcattgcgatagccaatggcttggggacagagtgatcacaacatccacccgcacgtgggccttgccaacatacaacaatcacctgtacaagcaaatcagtaactcaaccagcggtggaagcagtaatgacaacgcgtacttcggttactctaccccttggggatattttgacttcaaccgtttccactgccacttctcaccgagagactggcagcgcctcataaataacaactggggattccgccccaagcgactgaacttcaagttgttcaacatccaggttaaagaggtgactgacaacaatggtgtgaagacaatcgccaataacctcacgagtaccgtccaggtcttcactgacagtgattatcaactgccctacgtgcttggatctgctcacgagggatgcctgcccccattccccgctgacgttttcatgattcctcagtacggctatctgacactcaatgatggcagccaggcggtcggtaggtcctcattttactgcctcgaatatttcccttcacaaatgctgcgcacggggaacaacttccagttctcctacgagtttgagaacgtcccattccatagcagctacgctcactctcaatctctggacaggctcatgaatcctctcatcgaccaatacctgtactatttgagcaagacaattgacggcagtgggcaaaaccagcaaacacttaaattcagtgttgccggacctagtaacatggcggtacagggaaggaactacattccgggcccatcctaccgtcaacaacgggtgtccaccaccgtcactcaaaacaacaactccgaatttgcatggccaggagcctcaagctgggcacttaatggaaggaatagcctgatgaatccagggcctgcaatggctagtcacaaagagggagaggaccgcttctttccattgtccgggtctctcatctttggcaaacaaggtacaggacgtgacaacgtggatgccgacaaagtgatgattaccaacgaggaagaaattaaaactacaaaccccgttgcgacagagtcctatggtcaagtcgccaccaaccatcagtcagccggcggcggcggtagcggcggtggcggatcaggaggaggtgggtctggtggaggaggatctggcggagacatgtcacaggtgcagctggtggaatcaggtggtggtcgcgtgcagactggcgggtccctgcgcctttcttgtgcagctagtggcatttcattcagtataactacaatgtactggtacagacaggcaccaggtgagcagagacagctggtcgctcttattactgatcgcgggaacacctactatgtcgactcagtgaagggcaggttcaccatcagtagagacgacagtaagaacacggtctatttgcaaatgaacgacctgaaacctgaggacacggccgtgtatttctgtaatagtatcccaggaaacgactggggtcaggggacgcaggttacagtcagtagcgcggccgctggcgcccaggcacaggctcaaaccggttgggtgcaaaaccaaggcatcttgcctggcatggtttggcaggaccgcgatgtttatctccaaggacccatttgggccaaaattcctcacacggacgggaactttcacccatcacctctgatgggcggctttggcatgaagcatcccccaccccagatcctcatcaagaacacgcctgtacccgcagatcccccgaccgccttcaacaaggacaagctgaactccttcatcacacagtattccacagggcaagtctcagttgagatcgagtgggagctgcaaaaggaaaacagcaagcgctggaaccccgagatccagtacacgtcaaactattacaagtctaataatgtcgaatttgccgtgaatacggaaggtgtgtattccgaacctcggcccataggcactcggtacctgactagaaatttg

SEQ ID NO: 13 - protein, 1025 aa, synthetic construct
MAADGYLPDWLEDNLSEGIREWWALKPGAPQPKANQQHQDNARGLVLPGYKYLGPGNGLDKGEPVNAADAAALEHDKAYDQQLKAGDNPYLKYNHADAEFQERLKEDTSFGGNLGRAVFQAKKRLLEPLGLVEEAAKTAPGKKRPVEQSPQEPDSSAGIGKSGAQPAKKRLNFGQTGDTESVPDPQPIGEPPAAPSGVGSLTMASGGGAPVADNNEGADGVGSSSGNWHCDSQWLGDRVITTSTRTWALPTYNNHLYKQISNSTSGGSSNDNAYFGYSTPWGYFDFNRFHCHFSPRDWQRLINNNWGFRPKRLNFKLFNIQVKEVTDNNGVKTIANNLTSTVQVFTDSDYQLPYVLGSAHEGCLPPFPADVFMIPQYGYLTLNDGSQAVGRSSFYCLEYFPSQMLRTGNNFQFSYEFENVPFHSSYAHSQSLDRLMNPLIDQYLYYLSKTIDGAGGGGSGGGGSGGGGSGGGGSGGGGSDVQLQASGGGSVQAGGSLTLSCRYSGGFVFRVSSMGWYRQAPGNQRELIATITVGGKTNYKDSVQRFIISRNDTTVTLQMNRLQPEDTAVYYCNLASTAVGADTWGQGTRVTVSSGGGGAGQNQQTLKFSVAGPSNMAVQGRNYIPGPSYRQQRVSTTVTQNNNSEFAAPGASSWALNGRNSLMNPGPAMASHKEGEDRFFPLSGSLIFGKQGTGRDNVDADKVMITNEEEIKTTNPVATESYGQVATNHQSAGGGGSGGGGSGGGGSGGGGSGGDMSQVQLVETGGGLVQPGGSLRLSCTASGFTFSMHAMTWYRQAPGKQRELVAVITSHGDRANYTDSVRGRFTISRDNTKNMVYLQMNSLKPEDTAVYYCNVPRYDSWGQGTQVTVSSAAAGAQAQAQTGWVQNQGILPGMVWQDRDVYLQGPIWAKIPHTDGNFHPSPLMGGFGMKHPPPQILIKNTPVPADPPTAFNKDKLNSFITQYSTGQVSVEIEWELQKENSKRWNPEIQYTSNYYKSNNVEFAVNTEGVYSEPRPIGTRYLTRNL

SEQ ID NO: 14 - DNA, 3078 bp, synthetic construct
  source 1..3078: mol_type = other DNA
atggccgctgatggctatctacccgattggcttgaggacaacctgtccgaaggaatcagggagtggtgggcgttgaaaccaggagccccgcaaccgaaggccaatcaacaacatcaagacaacgcccggggacttgtcctgccaggctacaaatacttgggacccggcaacggactggacaagggcgagccagtaaacgcggctgacgcggcggctctggagcacgacaaggcctacgaccagcagttgaaggccggtgacaacccgtacctcaagtacaaccacgccgacgccgagttccaggagcggcttaaggaagatactagttttggcggaaacctcggtagggctgttttccaggccaagaagcggctgcttgaacccttgggcctggttgaggaagctgctaaaaccgccccaggaaagaaacgtccagtggagcagagtccccaggaaccagactcctcagctggtattggcaaaagtggcgcacaaccggctaagaagcgactcaatttcggccagaccggggatactgagtccgttcctgatccgcaacctattggagagccgcccgcggccccaagcggcgtgggctctttgactatggcttccggtggcggcgctcctgtggccgacaacaacgaaggagctgatggagtgggatcatcctcaggtaattggcattgcgatagccaatggcttggggacagagtgatcacaacatccacccgcacgtgggccttgccaacatacaacaatcacctgtacaagcaaatcagtaactcaaccagcggtggaagcagtaatgacaacgcgtacttcggttactctaccccttggggatattttgacttcaaccgtttccactgccacttctcaccgagagactggcagcgcctcataaataacaactggggattccgccccaagcgactgaacttcaagttgttcaacatccaggttaaagaggtgactgacaacaatggtgtgaagacaatcgccaataacctcacgagtaccgtccaggtcttcactgacagtgattatcaactgccctacgtgcttggatctgctcacgagggatgcctgcccccattccccgctgacgttttcatgattcctcagtacggctatctgacactcaatgatggcagccaggcggtcggtaggtcctcattttactgcctcgaatatttcccttcacaaatgctgcgcacggggaacaacttccagttctcctacgagtttgagaacgtcccattccatagcagctacgctcactctcaatctctggacaggctcatgaatcctctcatcgaccaatacctgtactatttgagcaagacaattgacggtgccggcggaggcggatctggcggaggcggaagtggcggcggaggaagcggagggggcggatctggggggggaggctcagatgtgcagctgcaggcgtctgggggaggctcggtgcaggctggagggtctctgacgctctcctgtagatactctggtggattcgtctttagagtcagtagtatgggctggtaccgccaggctccagggaaccagcgcgagttgatcgcaacgattactgttggcgggaaaacaaactataaagactccgtacagcgatttatcatctccagaaacgatacgacggtgacgctacagatgaatagactgcaacctgaggacacagccgtctattactgtaatttagcatcaacggcagttggagccgacacctggggccaggggacccgggtcaccgtctcctcaggaggtggaggcgccgggcaaaatcagcagacactcaaattctcagttgcagggccttctaacatggccgttcagggccgtaactacattccgggcccctcataccgacaacaacgcgtgagtactactgttacacaaaacaacaactccgaatttgctgcgccaggagcctcaagctgggctcttaatggtcgtaattccctgatgaatcctgggcccgcgatggccagtcacaaagagggcgaggaccgattctttccactcagcggaagcttgatctttggaaaacaagggacgggtcgcgacaacgttgatgccgacaaagttatgataaccaacgaggaagaaatcaaaacaacgaacccggttgctactgagtcttatggtcaagttgccaccaaccaccagtccgcgggcggcggcggtagcggcggtggcggatcaggaggaggtgggtctggtggaggaggatctggcggagacatgtcacaagtacaattagtggagacaggtggtggtctggtgcaacccggcggtagcctgaggttgagttgcacagcttccggctttaccttcagcatgcatgcaatgacttggtatagacaggccccaggaaaacaacgggagctggtcgccgtgatcacatcacacggtgaccgggccaattacacagattctgtcaggggacggttcaccatttcacgtgataatacaaagaatatggtttatctccaaatgaatagccttaaaccagaggataccgctgtgtattactgtaatgtcccacgatatgattcctggggccagggaacacaagtaaccgttagcagcgcggccgctggcgcgcaagcacaggctcagaccggttgggtgcaaaaccaaggcatcttgcctggcatggtttggcaggaccgcgatgtttatctccaaggacccatttgggccaaaattcctcacacggacgggaactttcacccatcacctctgatgggcggctttggcatgaagcatcccccaccccagatcctcatcaagaacacgcctgtacccgcagatcccccgaccgccttcaacaaggacaagctgaactccttcatcacacagtattccacagggcaagtctcagttgagatcgagtgggagctgcaaaaggaaaacagcaagcgctggaaccccgagatccagtacacgtcaaactattacaagtctaataatgtcgaatttgccgtgaatacggaaggtgtgtattccgaacctcggcccataggcactcggtacctgactagaaatttgtga

SEQ ID NO: 15 - protein, 882 aa, synthetic construct
MAADGYLPDWLEDTLSEGIRQWWKLKPGPPPPKPAERHKDDSRGLVLPGYKYLGPFNGLDKGEPVNEADAAALEHDKAYDRQLDSGDNPYLKYNHADAEFQERLKEDTSFGGNLGRAVFQAKKRVLEPLGLVEEPVKTAPTGKRIDDHFPKRKKARTEEDSKPSTSSDAEAGPSGSQQLQIPAQPASSLGADTMSAGGGGPLGDNNQGADGVGNASGDWHCDSTWMGDRVVTKSTRTWVLPSYNNHQYREIKSGSVDGSNANAYFGYSTPWGYFDFNRFHSHWSPRDWQRLINNYWGFRPRSLRVKIFNIQVKEVTVQDSTTTIANNLTSTVQVFTDDDYQLPYVVGNGTEGCLPAFPPQVFTLPQYGYATLNRDNTENPTERSSFFCLEYFPSKMLRTGNNFEFTYNFEEVPFHSSFAPSQNLFKLANPLVDQYLYRFVSTNAGGGGSGGGGSGGGGSGGGGSGGGGSDVQLQESGGGLVQAGDSLRLSCVGSGRRFDNYAMAWFRQAPGKERTFVAAISWSSGTTRYLDTVKGRFTISRDNAKSTVYLQMNSLKPEDTAVYYCAARYQPRYYDSGDMDGYEYEFWGQGTQVTVSSGGGGAGGVQFNKNLAGRYANTYKNWFPGPMGRTQGWNLGSGVNRASVSAFATTNRMELEGASYQVPPQPNGMTNNLQGSNTYALENTMIFNSQPANPGTTATYLEGNMLITSESETQPVNRVAYNVGGQMATNNQSSTTAPATGTYNLQEIVPGSVWMERDVYLQGPIWAKIPETGAHFHPSPAMGGFGLKHPPPMMLIKNTPVPGNITSFSDVPVSSFITQYSTGQVTVEMEWELKKENSKRWNPEIQYTNNYNDPQFVDFAPDSTGEYRTTRPIGTRYLTRPL

SEQ ID NO: 16 - DNA, 2646 bp, synthetic construct
  source 1..2646: mol_type = other DNA
atggctgccgatggttatctacccgattggctcgaggacactctctctgaaggaataagacagtggtggaagctcaaacctggcccaccaccaccaaagcccgcagagcggcataaggacgacagcaggggtcttgtgcttcctgggtacaagtacctcggacccttcaacggactcgacaagggagagccggtcaacgaggcagacgccgcggccctcgagcacgacaaagcctacgaccggcagctcgacagcggagacaacccgtacctcaagtacaaccacgccgacgcggagtttcaggagcgccttaaagaagatacgtcttttgggggcaacctcggacgagcagtcttccaggcgaaaaagagggttcttgaacctctgggcctggttgaggaacctgttaagacggcccctaccggaaagcggatagacgaccactttccaaaaagaaagaaggctcggaccgaagaggactccaagccttccacctcgtcagacgccgaagctggacccagcggatcccagcagctgcaaatcccagcccaaccagcctcaagtttgggagctgatacaatgtctgcgggaggtggcggcccattgggcgacaataaccaaggtgccgatggagtgggcaatgcctcgggagattggcattgcgattccacgtggatgggggacagagtcgtcaccaagtccacccgaacctgggtgctgcccagctacaacaaccaccagtaccgagagatcaaaagcggctccgtcgacggaagcaacgccaacgcctactttggatacagcaccccctgggggtactttgactttaaccgcttccacagccactggagcccccgagactggcaaagactcatcaacaactactggggcttcagaccccggtccctcagagtcaaaatcttcaacattcaagtcaaagaggtcacggtgcaggactccaccaccaccatcgccaacaacctcacctccaccgtccaagtgtttacggacgacgactaccagctgccctacgtcgtcggcaacgggaccgagggatgcctcccggccttccctccgcaggtctttacgctgccgcagtacggttacgcgacgctgaaccgcgacaacacagaaaatcccaccgagaggagcagcttcttctgcctagagtactttcccagcaagatgctgagaacgggcaacaactttgagtttacctacaactttgaggaggtgcccttccactccagcttcgctcccagtcagaacctgttcaagctggccaacccgctggtggaccagtacttgtaccgcttcgtgagcacaaatgccggcggaggcggatctggcggaggcggaagtggcggcggaggaagcggagggggcggatctggggggggaggctcagatgtacaactgcaagagagtggcggtgggctcgttcaagctggggatagcctgcgcctgtcatgcgtagggagtggcagacgctttgacaactacgcaatggcctggtttcgccaggcccctggaaaagaacggacttttgtggctgctatctcctggagtagcggaacgacgagatacctggatacagttaaaggtcgctttaccatttcacgcgacaatgccaagagtacagtgtacctgcaaatgaactctcttaaacccgaagacactgcagtgtactactgtgctgctcgttatcaacctcgctattatgactcaggagacatggacggctacgaatatgaattttggggacaaggtactcaagtcaccgtctccagtggaggtggaggcgccggaggagtccagttcaacaagaacctggccgggagatacgccaacacctacaaaaactggttcccggggcccatgggccgaacccagggctggaacctgggctccggggtcaaccgcgccagtgtcagcgccttcgccacgaccaataggatggagctcgagggcgcgagttaccaggtgcccccgcagccgaacggcatgaccaacaacctccagggcagcaacacctatgccctggagaacactatgatcttcaacagccagccagcgaacccgggcaccaccgccacgtacctcgagggcaacatgctcatcaccagcgagagcgagacgcagccggtgaaccgcgtggcgtacaacgtcggcgggcagatggccaccaacaaccagagctccaccactgcccccgcgaccggcacgtacaacctccaggaaatcgtgcccggcagcgtgtggatggagagggacgtgtacctccaaggacccatctgggccaagatcccagagacgggggcgcactttcacccctctccggccatgggcggattcggactcaaacacccaccgcccatgatgctcatcaagaacacgcctgtgcccggaaatatcaccagcttctcggacgtgcccgtcagcagcttcatcacccagtacagcaccgggcaggtcaccgtggagatggagtgggagctcaagaaggaaaactccaagaggtggaacccagagatccagtacacaaacaactacaacgacccccagtttgtggactttgccccggacagcaccggggaatacagaaccaccagacctatcggaacccgataccttacccgacccctt

SEQ ID NO: 17 - protein, 882 aa, synthetic construct
MAADGYLPDWLEDTLSEGIRQWWKLKPGPPPPKPAERHKDDSRGLVLPGYKYLGPFNGLDKGEPVNEADAAALEHDKAYDRQLDSGDNPYLKYNHADAEFQERLKEDTSFGGNLGRAVFQAKKRVLEPLGLVEEPVKTAPTGKRIDDHFPKRKKARTEEDSKPSTSSDAEAGPSGSQQLQIPAQPASSLGADTMSAGGGGPLGDNNQGADGVGNASGDWHCDSTWMGDRVVTKSTRTWVLPSYNNHQYREIKSGSVDGSNANAYFGYSTPWGYFDFNRFHSHWSPRDWQRLINNYWGFRPRSLRVKIFNIQVKEVTVQDSTTTIANNLTSTVQVFTDDDYQLPYVVGNGTEGCLPAFPPQVFTLPQYGYATLNRDNTENPTERSSFFCLEYFPSKMLRTGNNFEFTYNFEEVPFHSSFAPSQNLFKLANPLVDQYLYRFVSTNNTGGVQFNKNLAGRYANTYKNWFPGPMGRTQGWNLGSGVNRASVSAFATTNRMELEGASYQVPPQPNGMTNNLQGSNTYALENTMIFNSQPANPGTTATYLEGNMLITSESETQPVNRVAYNVGGQMATNNQSAGGGGSGGGGSGGGGSGGGGSGGGGSDVQLQESGGGLVQAGDSLRLSCVGSGRRFDNYAMAWFRQAPGKERTFVAAISWSSGTTRYLDTVKGRFTISRDNAKSTVYLQMNSLKPEDTAVYYCAARYQPRYYDSGDMDGYEYEFWGQGTQVTVSSGGGGATAPATGTYNLQEIVPGSVWMERDVYLQGPIWAKIPETGAHFHPSPAMGGFGLKHPPPMMLIKNTPVPGNITSFSDVPVSSFITQYSTGQVTVEMEWELKKENSKRWNPEIQYTNNYNDPQFVDFAPDSTGEYRTTRPIGTRYLTRPL

SEQ ID NO: 18 - DNA, 2646 bp, synthetic construct
  source 1..2646: mol_type = other DNA
atggctgccgatggttatctacccgattggctcgaggacactctctctgaaggaataagacagtggtggaagctcaaacctggcccaccaccaccaaagcccgcagagcggcataaggacgacagcaggggtcttgtgcttcctgggtacaagtacctcggacccttcaacggactcgacaagggagagccggtcaacgaggcagacgccgcggccctcgagcacgacaaagcctacgaccggcagctcgacagcggagacaacccgtacctcaagtacaaccacgccgacgcggagtttcaggagcgccttaaagaagatacgtcttttgggggcaacctcggacgagcagtcttccaggcgaaaaagagggttcttgaacctctgggcctggttgaggaacctgttaagacggcccctaccggaaagcggatagacgaccactttccaaaaagaaagaaggctcggaccgaagaggactccaagccttccacctcgtcagacgccgaagctggacccagcggatcccagcagctgcaaatcccagcccaaccagcctcaagtttgggagctgatacaatgtctgcgggaggtggcggcccattgggcgacaataaccaaggtgccgatggagtgggcaatgcctcgggagattggcattgcgattccacgtggatgggggacagagtcgtcaccaagtccacccgaacctgggtgctgcccagctacaacaaccaccagtaccgagagatcaaaagcggctccgtcgacggaagcaacgccaacgcctactttggatacagcaccccctgggggtactttgactttaaccgcttccacagccactggagcccccgagactggcaaagactcatcaacaactactggggcttcagaccccggtccctcagagtcaaaatcttcaacattcaagtcaaagaggtcacggtgcaggactccaccaccaccatcgccaacaacctcacctccaccgtccaagtgtttacggacgacgactaccagctgccctacgtcgtcggcaacgggaccgagggatgcctcccggccttccctccgcaggtctttacgctgccgcagtacggttacgcgacgctgaaccgcgacaacacagaaaatcccaccgagaggagcagcttcttctgcctagagtactttcccagcaagatgctgagaacgggcaacaactttgagtttacctacaactttgaggaggtgcccttccactccagcttcgctcccagtcagaacctgttcaagctggccaacccgctggtggaccagtacttgtaccgcttcgtgagcacaaataacactgggggagtccagttcaacaagaacctggccgggagatacgccaacacctacaaaaactggttcccggggcccatgggccgaacccagggctggaacctgggctccggggtcaaccgcgccagtgtcagcgccttcgccacgaccaataggatggagctcgagggcgcgagttaccaggtgcccccgcagccgaacggcatgaccaacaacctccagggcagcaacacctatgccctggagaacactatgatcttcaacagccagccagcgaacccgggcaccaccgccacgtacctcgagggcaacatgctcatcaccagcgagagcgagacgcagccggtgaaccgcgtggcgtacaacgtcggcgggcagatggccaccaacaaccagagcgccggcggaggcggatctggcggaggcggaagtggcggcggaggaagcggagggggcggatctggggggggaggctcagatgtacaactgcaagagagtggcggtgggctcgttcaagctggggatagcctgcgcctgtcatgcgtagggagtggcagacgctttgacaactacgcaatggcctggtttcgccaggcccctggaaaagaacggacttttgtggctgctatctcctggagtagcggaacgacgagatacctggatacagttaaaggtcgctttaccatttcacgcgacaatgccaagagtacagtgtacctgcaaatgaactctcttaaacccgaagacactgcagtgtactactgtgctgctcgttatcaacctcgctattatgactcaggagacatggacggctacgaatatgaattttggggacaaggtactcaagtcaccgtctccagtggaggtggaggcgccactgcccccgcgaccggcacgtacaacctccaggaaatcgtgcccggcagcgtgtggatggagagggacgtgtacctccaaggacccatctgggccaagatcccagagacgggggcgcactttcacccctctccggccatgggcggattcggactcaaacacccaccgcccatgatgctcatcaagaacacgcctgtgcccggaaatatcaccagcttctcggacgtgcccgtcagcagcttcatcacccagtacagcaccgggcaggtcaccgtggagatggagtgggagctcaagaaggaaaactccaagaggtggaacccagagatccagtacacaaacaactacaacgacccccagtttgtggactttgccccggacagcaccggggaatacagaaccaccagacctatcggaacccgataccttacccgacccctt

SEQ ID NO: 19 - protein, 736 aa, Adeno-associated virus serotype 1
MAADGYLPDWLEDNLSEGIREWWDLKPGAPKPKANQQKQDDGRGLVLPGYKYLGPFNGLDKGEPVNAADAAALEHDKAYDQQLKAGDNPYLRYNHADAEFQERLQEDTSFGGNLGRAVFQAKKRVLEPLGLVEEGAKTAPGKKRPVEQSPQEPDSSSGIGKTGQQPAKKRLNFGQTGDSESVPDPQPLGEPPATPAAVGPTTMASGGGAPMADNNEGADGVGNASGNWHCDSTWLGDRVITTSTRTWALPTYNNHLYKQISSASTGASNDNHYFGYSTPWGYFDFNRFHCHFSPRDWQRLINNNWGFRPKRLNFKLFNIQVKEVTTNDGVTTIANNLTSTVQVFSDSEYQLPYVLGSAHQGCLPPFPADVFMIPQYGYLTLNNGSQAVGRSSFYCLEYFPSQMLRTGNNFTFSYTFEEVPFHSSYAHSQSLDRLMNPLIDQYLYYLNRTQNQSGSAQNKDLLFSRGSPAGMSVQPKNWLPGPCYRQQRVSKTKTDNNNSNFTWTGASKYNLNGRESIINPGTAMASHKDDEDKFFPMSGVMIFGKESAGASNTALDNVMITDEEEIKATNPVATERFGTVAVNFQSSSTDPATGDVHAMGALPGMVWQDRDVYLQGPIWAKIPHTDGHFHPSPLMGGFGLKNPPPQILIKNTPVPANPPAEFSATKFASFITQYSTGQVSVEIEWELQKENSKRWNPEVQYTSNYAKSANVDFTVDNNGLYTEPRPIGTRYLTRPL

SEQ ID NO: 20 - protein, 599 aa, Adeno-associated virus serotype 1
TAPGKKRPVEQSPQEPDSSSGIGKTGQQPAKKRLNFGQTGDSESVPDPQPLGEPPATPAAVGPTTMASGGGAPMADNNEGADGVGNASGNWHCDSTWLGDRVITTSTRTWALPTYNNHLYKQISSASTGASNDNHYFGYSTPWGYFDFNRFHCHFSPRDWQRLINNNWGFRPKRLNFKLFNIQVKEVTTNDGVTTIANNLTSTVQVFSDSEYQLPYVLGSAHQGCLPPFPADVFMIPQYGYLTLNNGSQAVGRSSFYCLEYFPSQMLRTGNNFTFSYTFEEVPFHSSYAHSQSLDRLMNPLIDQYLYYLNRTQNQSGSAQNKDLLFSRGSPAGMSVQPKNWLPGPCYRQQRVSKTKTDNNNSNFTWTGASKYNLNGRESIINPGTAMASHKDDEDKFFPMSGVMIFGKESAGASNTALDNVMITDEEEIKATNPVATERFGTVAVNFQSSSTDPATGDVHAMGALPGMVWQDRDVYLQGPIWAKIPHTDGHFHPSPLMGGFGLKNPPPQILIKNTPVPANPPAEFSATKFASFITQYSTGQVSVEIEWELQKENSKRWNPEVQYTSNYAKSANVDFTVDNNGLYTEPRPIGTRYLTRPL

SEQ ID NO: 21 - protein, 534 aa, Adeno-associated virus serotype 1
MASGGGAPMADNNEGADGVGNASGNWHCDSTWLGDRVITTSTRTWALPTYNNHLYKQISSASTGASNDNHYFGYSTPWGYFDFNRFHCHFSPRDWQRLINNNWGFRPKRLNFKLFNIQVKEVTTNDGVTTIANNLTSTVQVFSDSEYQLPYVLGSAHQGCLPPFPADVFMIPQYGYLTLNNGSQAVGRSSFYCLEYFPSQMLRTGNNFTFSYTFEEVPFHSSYAHSQSLDRLMNPLIDQYLYYLNRTQNQSGSAQNKDLLFSRGSPAGMSVQPKNWLPGPCYRQQRVSKTKTDNNNSNFTWTGASKYNLNGRESIINPGTAMASHKDDEDKFFPMSGVMIFGKESAGASNTALDNVMITDEEEIKATNPVATERFGTVAVNFQSSSTDPATGDVHAMGALPGMVWQDRDVYLQGPIWAKIPHTDGHFHPSPLMGGFGLKNPPPQILIKNTPVPANPPAEFSATKFASFITQYSTGQVSVEIEWELQKENSKRWNPEVQYTSNYAKSANVDFTVDNNGLYTEPRPIGTRYLTRPL

SEQ ID NO: 22 - protein, 735 aa, Adeno-associated virus serotype 2 [sequence omitted]

SEQ ID NO: 23 - protein, 598 aa, Adeno-associated virus serotype 2
TAPGKKRPVEHSPVEPDSSSGTGKAGQQPARKRLNFGQTGDADSVPDPQPLGQPPAAPSGLGTNTMATGSGAPMADNNEGADGVGNSSGNWHCDSTWMGDRVITTSTRTWALPTYNNHLYKQISSQSGASNDNHYFGYSTPWGYFDFNRFHCHFSPRDWQRLINNNWGFRPKRLNFKLFNIQVKEVTQNDGTTTIANNLTSTVQVFTDSEYQLPYVLGSAHQGCLPPFPADVFMVPQYGYLTLNNGSQAVGRSSFYCLEYFPSQMLRTGNNFTFSYTFEDVPFHSSYAHSQSLDRLMNPLIDQYLYYLSRTNTPSGTTTQSRLQFSQAGASDIRDQSRNWLPGPCYRQQRVSKTSADNNNSEYSWTGATKYHLNGRDSLVNPGPAMASHKDDEEKFFPQSGVLIFGKQGSEKTNVDIEKVMITDEEEIRTTNPVATEQYGSVSTNLQRGNRQAATADVNTQGVLPGMVWQDRDVYLQGPIWAKIPHTDGHFHPSPLMGGFGLKHPPPQILIKNTPVPANPSTTFSAAKFASFITQYSTGQVSVEIEWELQKENSKRWNPEIQYTSNYNKSVNVDFTVDTNGVYSEPRPIGTRYLTRNL

SEQ ID NO: 24 - protein, 533 aa, Adeno-associated virus serotype 2
MATGSGAPMADNNEGADGVGNSSGNWHCDSTWMGDRVITTSTRTWALPTYNNHLYKQISSQSGASNDNHYFGYSTPWGYFDFNRFHCHFSPRDWQRLINNNWGFRPKRLNFKLFNIQVKEVTQNDGTTTIANNLTSTVQVFTDSEYQLPYVLGSAHQGCLPPFPADVFMVPQYGYLTLNNGSQAVGRSSFYCLEYFPSQMLRTGNNFTFSYTFEDVPFHSSYAHSQSLDRLMNPLIDQYLYYLSRTNTPSGTTTQSRLQFSQAGASDIRDQSRNWLPGPCYRQQRVSKTSADNNNSEYSWTGATKYHLNGRDSLVNPGPAMASHKDDEEKFFPQSGVLIFGKQGSEKTNVDIEKVMITDEEEIRTTNPVATEQYGSVSTNLQRGNRQAATADVNTQGVLPGMVWQDRDVYLQGPIWAKIPHTDGHFHPSPLMGGFGLKHPPPQILIKNTPVPANPSTTFSAAKFASFITQYSTGQVSVEIEWELQKENSKRWNPEIQYTSNYNKSVNVDFTVDTNGVYSEPRPIGTRYLTRNL

SEQ ID NO: 25 - protein, 736 aa, Adeno-associated virus serotype 3
MAADGYLPDWLEDNLSEGIREWWALKPGVPQPKANQQHQDNRRGLVLPGYKYLGPGNGLDKGEPVNEADAAALEHDKAYDQQLKAGDNPYLKYNHADAEFQERLQEDTSFGGNLGRAVFQAKKRILEPLGLVEEAAKTAPGKKGAVDQSPQEPDSSSGVGKSGKQPARKRLNFGQTGDSESVPDPQPLGEPPAAPTSLGSNTMASGGGAPMADNNEGADGVGNSSGNWHCDSQWLGDRVITTSTRTWALPTYNNHLYKQISSQSGASNDNHYFGYSTPWGYFDFNRFHCHFSPRDWQRLINNNWGFRPKKLSFKLFNIQVRGVTQNDGTTTIANNLTSTVQVFTDSEYQLPYVLGSAHQGCLPPFPADVFMVPQYGYLTLNNGSQAVGRSSFYCLEYFPSQMLRTGNNFQFSYTFEDVPFHSSYAHSQSLDRLMNPLIDQYLYYLNRTQGTTSGTTNQSRLLFSQAGPQSMSLQARNWLPGPCYRQQRLSKTANDNNNSNFPWTAASKYHLNGRDSLVNPGPAMASHKDDEEKFFPMHGNLIFGKEGTTASNAELDNVMITDEEEIRTTNPVATEQYGTVANNLQSSNTAPTTGTVNHQGALPGMVWQDRDVYLQGPIWAKIPHTDGHFHPSPLMGGFGLKHPPPQIMIKNTPVPANPPTTFSPAKFASFITQYSTGQVSVEIEWELQKENSKRWNPEIQYTSNYNKSVNVDFTVDTNGVYSEPRPIGTRYLTRNL

SEQ ID NO: 26 - protein, 599 aa, Adeno-associated virus serotype 3
TAPGKKGAVDQSPQEPDSSSGVGKSGKQPARKRLNFGQTGDSESVPDPQPLGEPPAAPTSLGSNTMASGGGAPMADNNEGADGVGNSSGNWHCDSQWLGDRVITTSTRTWALPTYNNHLYKQISSQSGASNDNHYFGYSTPWGYFDFNRFHCHFSPRDWQRLINNNWGFRPKKLSFKLFNIQVRGVTQNDGTTTIANNLTSTVQVFTDSEYQLPYVLGSAHQGCLPPFPADVFMVPQYGYLTLNNGSQAVGRSSFYCLEYFPSQMLRTGNNFQFSYTFEDVPFHSSYAHSQSLDRLMNPLIDQYLYYLNRTQGTTSGTTNQSRLLFSQAGPQSMSLQARNWLPGPCYRQQRLSKTANDNNNSNFPWTAASKYHLNGRDSLVNPGPAMASHKDDEEKFFPMHGNLIFGKEGTTASNAELDNVMITDEEEIRTTNPVATEQYGTVANNLQSSNTAPTTGTVNHQGALPGMVWQDRDVYLQGPIWAKIPHTDGHFHPSPLMGGFGLKHPPPQIMIKNTPVPANPPTTFSPAKFASFITQYSTGQVSVEIEWELQKENSKRWNPEIQYTSNYNKSVNVDFTVDTNGVYSEPRPIGTRYLTRNL

SEQ ID NO: 27 - protein, 534 aa, Adeno-associated virus serotype 3
MASGGGAPMADNNEGADGVGNSSGNWHCDSQWLGDRVITTSTRTWALPTYNNHLYKQISSQSGASNDNHYFGYSTPWGYFDFNRFHCHFSPRDWQRLINNNWGFRPKKLSFKLFNIQVRGVTQNDGTTTIANNLTSTVQVFTDSEYQLPYVLGSAHQGCLPPFPADVFMVPQYGYLTLNNGSQAVGRSSFYCLEYFPSQMLRTGNNFQFSYTFEDVPFHSSYAHSQSLDRLMNPLIDQYLYYLNRTQGTTSGTTNQSRLLFSQAGPQSMSLQARNWLPGPCYRQQRLSKTANDNNNSNFPWTAASKYHLNGRDSLVNPGPAMASHKDDEEKFFPMHGNLIFGKEGTTASNAELDNVMITDEEEIRTTNPVATEQYGTVANNLQSSNTAPTTGTVNHQGALPGMVWQDRDVYLQGPIWAKIPHTDGHFHPSPLMGGFGLKHPPPQIMIKNTPVPANPPTTFSPAKFASFITQYSTGQVSVEIEWELQKENSKRWNPEIQYTSNYNKSVNVDFTVDTNGVYSEPRPIGTRYLTRNL

SEQ ID NO: 28 - protein, 734 aa, Adeno-associated virus serotype 4
MTDGYLPDWLEDNLSEGVREWWALQPGAPKPKANQQHQDNARGLVLPGYKYLGPGNGLDKGEPVNAADAAALEHDKAYDQQLKAGDNPYLKYNHADAEFQQRLQGDTSFGGNLGRAVFQAKKRVLEPLGLVEQAGETAPGKKRPLIESPQQPDSSTGIGKKGKQPAKKKLVFEDETGAGDGPPEGSTSGAMSDDSEMRAAAGGAAVEGGQGADGVGNASGDWHCDSTWSEGHVTTTSTRTWVLPTYNNHLYKRLGESLQSNTYNGFSTPWGYFDFNRFHCHFSPRDWQRLINNNWGMRPKAMRVKIFNIQVKEVTTSNGETTVANNLTSTVQIFADSSYELPYVMDAGQEGSLPPFPNDVFMVPQYGYCGLVTGNTSQQQTDRNAFYCLEYFPSQMLRTGNNFEITYSFEKVPFHSMYAHSQSLDRLMNPLIDQYLWGLQSTTTGTTLNAGTATTNFTKLRPTNFSNFKKNWLPGPSIKQQGFSKTANQNYKIPATGSDSLIKYETHSTLDGRWSALTPGPPMATAGPADSKFSNSQLIFAGPKQNGNTATVPGTLIFTSEEELAATNATDTDMWGNLPGGDQSNSNLPTVDRLTALGAVPGMVWQNRDIYYQGPIWAKIPHTDGHFHPSPLIGGFGLKHPPPQIFIKNTPVPANPATTFSSTPVNSFITQYSTGQVSVQIDWEIQKERSKRWNPEVQFTSNYGQQNSLLWAPDAAGKYTEPRAIGTRYLTHHL

SEQ ID NO: 29 - protein, 598 aa, Adeno-associated virus serotype 4
TAPGKKRPLIESPQQPDSSTGIGKKGKQPAKKKLVFEDETGAGDGPPEGSTSGAMSDDSEMRAAAGGAAVEGGQGADGVGNASGDWHCDSTWSEGHVTTTSTRTWVLPTYNNHLYKRLGESLQSNTYNGFSTPWGYFDFNRFHCHFSPRDWQRLINNNWGMRPKAMRVKIFNIQVKEVTTSNGETTVANNLTSTVQIFADSSYELPYVMDAGQEGSLPPFPNDVFMVPQYGYCGLVTGNTSQQQTDRNAFYCLEYFPSQMLRTGNNFEITYSFEKVPFHSMYAHSQSLDRLMNPLIDQYLWGLQSTTTGTTLNAGTATTNFTKLRPTNFSNFKKNWLPGPSIKQQGFSKTANQNYKIPATGSDSLIKYETHSTLDGRWSALTPGPPMATAGPADSKFSNSQLIFAGPKQNGNTATVPGTLIFTSEEELAATNATDTDMWGNLPGGDQSNSNLPTVDRLTALGAVPGMVWQNRDIYYQGPIWAKIPHTDGHFHPSPLIGGFGLKHPPPQIFIKNTPVPANPATTFSSTPVNSFITQYSTGQVSVQIDWEIQKERSKRWNPEVQFTSNYGQQNSLLWAPDAAGKYTEPRAIGTRYLTHHL

SEQ ID NO: 30 - protein, 538 aa, Adeno-associated virus serotype 4
MRAAAGGAAVEGGQGADGVGNASGDWHCDSTWSEGHVTTTSTRTWVLPTYNNHLYKRLGESLQSNTYNGFSTPWGYFDFNRFHCHFSPRDWQRLINNNWGMRPKAMRVKIFNIQVKEVTTSNGETTVANNLTSTVQIFADSSYELPYVMDAGQEGSLPPFPNDVFMVPQYGYCGLVTGNTSQQQTDRNAFYCLEYFPSQMLRTGNNFEITYSFEKVPFHSMYAHSQSLDRLMNPLIDQYLWGLQSTTTGTTLNAGTATTNFTKLRPTNFSNFKKNWLPGPSIKQQGFSKTANQNYKIPATGSDSLIKYETHSTLDGRWSALTPGPPMATAGPADSKFSNSQLIFAGPKQNGNTATVPGTLIFTSEEELAATNATDTDMWGNLPGGDQSNSNLPTVDRLTALGAVPGMVWQNRDIYYQGPIWAKIPHTDGHFHPSPLIGGFGLKHPPPQIFIKNTPVPANPATTFSSTPVNSFITQYSTGQVSVQIDWEIQKERSKRWNPEVQFTSNYGQQNSLLWAPDAAGKYTEPRAIGTRYLTHHL

SEQ ID NO: 31 - protein, 724 aa, Adeno-associated virus serotype 5
MSFVDHPPDWLEEVGEGLREFLGLEAGPPKPKPNQQHQDQARGLVLPGYNYLGPGNGLDRGEPVNRADEVAREHDISYNEQLEAGDNPYLKYNHADAEFQEKLADDTSFGGNLGKAVFQAKKRVLEPFGLVEEGAKTAPTGKRIDDHFPKRKKARTEEDSKPSTSSDAEAGPSGSQQLQIPAQPASSLGADTMSAGGGGPLGDNNQGADGVGNASGDWHCDSTWMGDRVVTKSTRTWVLPSYNNHQYREIKSGSVDGSNANAYFGYSTPWGYFDFNRFHSHWSPRDWQRLINNYWGFRPRSLRVKIFNIQVKEVTVQDSTTTIANNLTSTVQVFTDDDYQLPYVVGNGTEGCLPAFPPQVFTLPQYGYATLNRDNTENPTERSSFFCLEYFPSKMLRTGNNFEFTYNFEEVPFHSSFAPSQNLFKLANPLVDQYLYRFVSTNNTGGVQFNKNLAGRYANTYKNWFPGPMGRTQGWNLGSGVNRASVSAFATTNRMELEGASYQVPPQPNGMTNNLQGSNTYALENTMIFNSQPANPGTTATYLEGNMLITSESETQPVNRVAYNVGGQMATNNQSSTTAPATGTYNLQEIVPGSVWMERDVYLQGPIWAKIPETGAHFHPSPAMGGFGLKHPPPMMLIKNTPVPGNITSFSDVPVSSFITQYSTGQVTVEMEWELKKENSKRWNPEIQYTNNYNDPQFVDFAPDSTGEYRTTRPIGTRYLTRPL

SEQ ID NO: 32 - protein, 588 aa, Adeno-associated virus serotype 5
TAPTGKRIDDHFPKRKKARTEEDSKPSTSSDAEAGPSGSQQLQIPAQPASSLGADTMSAGGGGPLGDNNQGADGVGNASGDWHCDSTWMGDRVVTKSTRTWVLPSYNNHQYREIKSGSVDGSNANAYFGYSTPWGYFDFNRFHSHWSPRDWQRLINNYWGFRPRSLRVKIFNIQVKEVTVQDSTTTIANNLTSTVQVFTDDDYQLPYVVGNGTEGCLPAFPPQVFTLPQYGYATLNRDNTENPTERSSFFCLEYFPSKMLRTGNNFEFTYNFEEVPFHSSFAPSQNLFKLANPLVDQYLYRFVSTNNTGGVQFNKNLAGRYANTYKNWFPGPMGRTQGWNLGSGVNRASVSAFATTNRMELEGASYQVPPQPNGMTNNLQGSNTYALENTMIFNSQPANPGTTATYLEGNMLITSESETQPVNRVAYNVGGQMATNNQSSTTAPATGTYNLQEIVPGSVWMERDVYLQGPIWAKIPETGAHFHPSPAMGGFGLKHPPPMMLIKNTPVPGNITSFSDVPVSSFITQYSTGQVTVEMEWELKKENSKRWNPEIQYTNNYNDPQFVDFAPDSTGEYRTTRPIGTRYLTRPL

SEQ ID NO: 33 - protein, 532 aa, Adeno-associated virus serotype 5
MSAGGGGPLGDNNQGADGVGNASGDWHCDSTWMGDRVVTKSTRTWVLPSYNNHQYREIKSGSVDGSNANAYFGYSTPWGYFDFNRFHSHWSPRDWQRLINNYWGFRPRSLRVKIFNIQVKEVTVQDSTTTIANNLTSTVQVFTDDDYQLPYVVGNGTEGCLPAFPPQVFTLPQYGYATLNRDNTENPTERSSFFCLEYFPSKMLRTGNNFEFTYNFEEVPFHSSFAPSQNLFKLANPLVDQYLYRFVSTNNTGGVQFNKNLAGRYANTYKNWFPGPMGRTQGWNLGSGVNRASVSAFATTNRMELEGASYQVPPQPNGMTNNLQGSNTYALENTMIFNSQPANPGTTATYLEGNMLITSESETQPVNRVAYNVGGQMATNNQSSTTAPATGTYNLQEIVPGSVWMERDVYLQGPIWAKIPETGAHFHPSPAMGGFGLKHPPPMMLIKNTPVPGNITSFSDVPVSSFITQYSTGQVTVEMEWELKKENSKRWNPEIQYTNNYNDPQFVDFAPDSTGEYRTTRPIGTRYLTRPL

SEQ ID NO: 34 - protein, 736 aa, Adeno-associated virus serotype 6
MAADGYLPDWLEDNLSEGIREWWDLKPGAPKPKANQQKQDDGRGLVLPGYKYLGPFNGLDKGEPVNAADAAALEHDKAYDQQLKAGDNPYLRYNHADAEFQERLQEDTSFGGNLGRAVFQAKKRVLEPFGLVEEGAKTAPGKKRPVEQSPQEPDSSSGIGKTGQQPAKKRLNFGQTGDSESVPDPQPLGEPPATPAAVGPTTMASGGGAPMADNNEGADGVGNASGNWHCDSTWLGDRVITTSTRTWALPTYNNHLYKQISSASTGASNDNHYFGYSTPWGYFDFNRFHCHFSPRDWQRLINNNWGFRPKRLNFKLFNIQVKEVTTNDGVTTIANNLTSTVQVFSDSEYQLPYVLGSAHQGCLPPFPADVFMIPQYGYLTLNNGSQAVGRSSFYCLEYFPSQMLRTGNNFTFSYTFEDVPFHSSYAHSQSLDRLMNPLIDQYLYYLNRTQNQSGSAQNKDLLFSRGSPAGMSVQPKNWLPGPCYRQQRVSKTKTDNNNSNFTWTGASKYNLNGRESIINPGTAMASHKDDKDKFFPMSGVMIFGKESAGASNTALDNVMITDEEEIKATNPVATERFGTVAVNLQSSSTDPATGDVHVMGALPGMVWQDRDVYLQGPIWAKIPHTDGHFHPSPLMGGFGLKHPPPQILIKNTPVPANPPAEFSATKFASFITQYSTGQVSVEIEWELQKENSKRWNPEVQYTSNYAKSANVDFTVDNNGLYTEPRPIGTRYLTRPL

SEQ ID NO: 35 - protein, 599 aa, Adeno-associated virus serotype 6
TAPGKKRPVEQSPQEPDSSSGIGKTGQQPAKKRLNFGQTGDSESVPDPQPLGEPPATPAAVGPTTMASGGGAPMADNNEGADGVGNASGNWHCDSTWLGDRVITTSTRTWALPTYNNHLYKQISSASTGASNDNHYFGYSTPWGYFDFNRFHCHFSPRDWQRLINNNWGFRPKRLNFKLFNIQVKEVTTNDGVTTIANNLTSTVQVFSDSEYQLPYVLGSAHQGCLPPFPADVFMIPQYGYLTLNNGSQAVGRSSFYCLEYFPSQMLRTGNNFTFSYTFEDVPFHSSYAHSQSLDRLMNPLIDQYLYYLNRTQNQSGSAQNKDLLFSRGSPAGMSVQPKNWLPGPCYRQQRVSKTKTDNNNSNFTWTGASKYNLNGRESIINPGTAMASHKDDKDKFFPMSGVMIFGKESAGASNTALDNVMITDEEEIKATNPVATERFGTVAVNLQSSSTDPATGDVHVMGALPGMVWQDRDVYLQGPIWAKIPHTDGHFHPSPLMGGFGLKHPPPQILIKNTPVPANPPAEFSATKFASFITQYSTGQVSVEIEWELQKENSKRWNPEVQYTSNYAKSANVDFTVDNNGLYTEPRPIGTRYLTRPL

SEQ ID NO: 36 - protein, 534 aa, Adeno-associated virus serotype 6
MASGGGAPMADNNEGADGVGNASGNWHCDSTWLGDRVITTSTRTWALPTYNNHLYKQISSASTGASNDNHYFGYSTPWGYFDFNRFHCHFSPRDWQRLINNNWGFRPKRLNFKLFNIQVKEVTTNDGVTTIANNLTSTVQVFSDSEYQLPYVLGSAHQGCLPPFPADVFMIPQYGYLTLNNGSQAVGRSSFYCLEYFPSQMLRTGNNFTFSYTFEDVPFHSSYAHSQSLDRLMNPLIDQYLYYLNRTQNQSGSAQNKDLLFSRGSPAGMSVQPKNWLPGPCYRQQRVSKTKTDNNNSNFTWTGASKYNLNGRESIINPGTAMASHKDDKDKFFPMSGVMIFGKESAGASNTALDNVMITDEEEIKATNPVATERFGTVAVNLQSSSTDPATGDVHVMGALPGMVWQDRDVYLQGPIWAKIPHTDGHFHPSPLMGGFGLKHPPPQILIKNTPVPANPPAEFSATKFASFITQYSTGQVSVEIEWELQKENSKRWNPEVQYTSNYAKSANVDFTVDNNGLYTEPRPIGTRYLTRPL

SEQ ID NO: 37 - protein, 737 aa, Adeno-associated virus serotype 7
MAADGYLPDWLEDNLSEGIREWWDLKPGAPKPKANQQKQDNGRGLVLPGYKYLGPFNGLDKGEPVNAADAAALEHDKAYDQQLKAGDNPYLRYNHADAEFQERLQEDTSFGGNLGRAVFQAKKRVLEPLGLVEEGAKTAPAKKRPVEPSPQRSPDSSTGIGKKGQQPARKRLNFGQTGDSESVPDPQPLGEPPAAPSSVGSGTVAAGGGAPMADNNEGADGVGNASGNWHCDSTWLGDRVITTSTRTWALPTYNNHLYKQISSETAGSTNDNTYFGYSTPWGYFDFNRFHCHFSPRDWQRLINNNWGFRPKKLRFKLFNIQVKEVTTNDGVTTIANNLTSTIQVFSDSEYQLPYVLGSAHQGCLPPFPADVFMIPQYGYLTLNNGSQSVGRSSFYCLEYFPSQMLRTGNNFEFSYSFEDVPFHSSYAHSQSLDRLMNPLIDQYLYYLARTQSNPGGTAGNRELQFYQGGPSTMAEQAKNWLPGPCFRQQRVSKTLDQNNNSNFAWTGATKYHLNGRNSLVNPGVAMATHKDDEDRFFPSSGVLIFGKTGATNKTTLENVLMTNEEEIRPTNPVATEEYGIVSSNLQAANTAAQTQVVNNQGALPGMVWQNRDVYLQGPIWAKIPHTDGNFHPSPLMGGFGLKHPPPQILIKNTPVPANPPEVFTPAKFASFITQYSTGQVSVEIEWELQKENSKRWNPEIQYTSNFEKQTGVDFAVDSQGVYSEPRPIGTRYLTRNL

SEQ ID NO: 38 - protein, 600 aa, Adeno-associated virus serotype 7
TAPAKKRPVEPSPQRSPDSSTGIGKKGQQPARKRLNFGQTGDSESVPDPQPLGEPPAAPSSVGSGTVAAGGGAPMADNNEGADGVGNASGNWHCDSTWLGDRVITTSTRTWALPTYNNHLYKQISSETAGSTNDNTYFGYSTPWGYFDFNRFHCHFSPRDWQRLINNNWGFRPKKLRFKLFNIQVKEVTTNDGVTTIANNLTSTIQVFSDSEYQLPYVLGSAHQGCLPPFPADVFMIPQYGYLTLNNGSQSVGRSSFYCLEYFPSQMLRTGNNFEFSYSFEDVPFHSSYAHSQSLDRLMNPLIDQYLYYLARTQSNPGGTAGNRELQFYQGGPSTMAEQAKNWLPGPCFRQQRVSKTLDQNNNSNFAWTGATKYHLNGRNSLVNPGVAMATHKDDEDRFFPSSGVLIFGKTGATNKTTLENVLMTNEEEIRPTNPVATEEYGIVSSNLQAANTAAQTQVVNNQGALPGMVWQNRDVYLQGPIWAKIPHTDGNFHPSPLMGGFGLKHPPPQILIKNTPVPANPPEVFTPAKFASFITQYSTGQVSVEIEWELQKENSKRWNPEIQYTSNFEKQTGVDFAVDSQGVYSEPRPIGTRYLTRNL

SEQ ID NO: 39 - protein, 534 aa, Adeno-associated virus serotype 7
VAAGGGAPMADNNEGADGVGNASGNWHCDSTWLGDRVITTSTRTWALPTYNNHLYKQISSETAGSTNDNTYFGYSTPWGYFDFNRFHCHFSPRDWQRLINNNWGFRPKKLRFKLFNIQVKEVTTNDGVTTIANNLTSTIQVFSDSEYQLPYVLGSAHQGCLPPFPADVFMIPQYGYLTLNNGSQSVGRSSFYCLEYFPSQMLRTGNNFEFSYSFEDVPFHSSYAHSQSLDRLMNPLIDQYLYYLARTQSNPGGTAGNRELQFYQGGPSTMAEQAKNWLPGPCFRQQRVSKTLDQNNNSNFAWTGATKYHLNGRNSLVNPGVAMATHKDDEDRFFPSSGVLIFGKTGATNKTTLENVLMTNEEEIRPTNPVATEEYGIVSSNLQAANTAAQTQVVNNQGALPGMVWQNRDVYLQGPIWAKIPHTDGNFHPSPLMGGFGLKHPPPQILIKNTPVPANPPEVFTPAKFASFITQYSTGQVSVEIEWELQKENSKRWNPEIQYTSNFEKQTGVDFAVDSQGVYSEPRPIGTRYLTRNL

SEQ ID NO: 40 - protein, 738 aa, Adeno-associated virus serotype 8
MAADGYLPDWLEDNLSEGIREWWALKPGAPKPKANQQKQDDGRGLVLPGYKYLGPFNGLDKGEPVNAADAAALEHDKAYDQQLQAGDNPYLRYNHADAEFQERLQEDTSFGGNLGRAVFQAKKRVLEPLGLVEEGAKTAPGKKRPVEPSPQRSPDSSTGIGKKGQQPARKRLNFGQTGDSESVPDPQPLGEPPAAPSGVGPNTMAAGGGAPMADNNEGADGVGSSSGNWHCDSTWLGDRVITTSTRTWALPTYNNHLYKQISNGTSGGATNDNTYFGYSTPWGYFDFNRFHCHFSPRDWQRLINNNWGFRPKRLSFKLFNIQVKEVTQNEGTKTIANNLTSTIQVFTDSEYQLPYVLGSAHQGCLPPFPADVFMIPQYGYLTLNNGSQAVGRSSFYCLEYFPSQMLRTGNNFQFTYTFEDVPFHSSYAHSQSLDRLMNPLIDQYLYYLSRTQTTGGTANTQTLGFSQGGPNTMANQAKNWLPGPCYRQQRVSTTTGQNNNSNFAWTAGTKYHLNGRNSLANPGIAMATHKDDEERFFPSNGILIFGKQNAARDNADYSDVMLTSEEEIKTTNPVATEEYGIVADNLQQQNTAPQIGTVNSQGALPGMVWQNRDVYLQGPIWAKIPHTDGNFHPSPLMGGFGLKHPPPQILIKNTPVPADPPTTFNQSKLNSFITQYSTGQVSVEIEWELQKENSKRWNPEIQYTSNYYKSTSVDFAVNTEGVYSEPRPIGTRYLTRNL

SEQ ID NO: 41 - protein, 601 aa, Adeno-associated virus serotype 8
TAPGKKRPVEPSPQRSPDSSTGIGKKGQQPARKRLNFGQTGDSESVPDPQPLGEPPAAPSGVGPNTMAAGGGAPMADNNEGADGVGSSSGNWHCDSTWLGDRVITTSTRTWALPTYNNHLYKQISNGTSGGATNDNTYFGYSTPWGYFDFNRFHCHFSPRDWQRLINNNWGFRPKRLSFKLFNIQVKEVTQNEGTKTIANNLTSTIQVFTDSEYQLPYVLGSAHQGCLPPFPADVFMIPQYGYLTLNNGSQAVGRSSFYCLEYFPSQMLRTGNNFQFTYTFEDVPFHSSYAHSQSLDRLMNPLIDQYLYYLSRTQTTGGTANTQTLGFSQGGPNTMANQAKNWLPGPCYRQQRVSTTTGQNNNSNFAWTAGTKYHLNGRNSLANPGIAMATHKDDEERFFPSNGILIFGKQNAARDNADYSDVMLTSEEEIKTTNPVATEEYGIVADNLQQQNTAPQIGTVNSQGALPGMVWQNRDVYLQGPIWAKIPHTDGNFHPSPLMGGFGLKHPPPQILIKNTPVPADPPTTFNQSKLNSFITQYSTGQVSVEIEWELQKENSKRWNPEIQYTSNYYKSTSVDFAVNTEGVYSEPRPIGTRYLTRNL

SEQ ID NO: 42 - protein, 535 aa, Adeno-associated virus serotype 8
MAAGGGAPMADNNEGADGVGSSSGNWHCDSTWLGDRVITTSTRTWALPTYNNHLYKQISNGTSGGATNDNTYFGYSTPWGYFDFNRFHCHFSPRDWQRLINNNWGFRPKRLSFKLFNIQVKEVTQNEGTKTIANNLTSTIQVFTDSEYQLPYVLGSAHQGCLPPFPADVFMIPQYGYLTLNNGSQAVGRSSFYCLEYFPSQMLRTGNNFQFTYTFEDVPFHSSYAHSQSLDRLMNPLIDQYLYYLSRTQTTGGTANTQTLGFSQGGPNTMANQAKNWLPGPCYRQQRVSTTTGQNNNSNFAWTAGTKYHLNGRNSLANPGIAMATHKDDEERFFPSNGILIFGKQNAARDNADYSDVMLTSEEEIKTTNPVATEEYGIVADNLQQQNTAPQIGTVNSQGALPGMVWQNRDVYLQGPIWAKIPHTDGNFHPSPLMGGFGLKHPPPQILIKNTPVPADPPTTFNQSKLNSFITQYSTGQVSVEIEWELQKENSKRWNPEIQYTSNYYKSTSVDFAVNTEGVYSEPRPIGTRYLTRNL

SEQ ID NO: 43 - protein, 736 aa, Adeno-associated virus serotype 9
MAADGYLPDWLEDNLSEGIREWWALKPGAPQPKANQQHQDNARGLVLPGYKYLGPGNGLDKGEPVNAADAAALEHDKAYDQQLKAGDNPYLKYNHADAEFQERLKEDTSFGGNLGRAVFQAKKRLLEPLGLVEEAAKTAPGKKRPVEQSPQEPDSSAGIGKSGAQPAKKRLNFGQTGDTESVPDPQPIGEPPAAPSGVGSLTMASGGGAPVADNNEGADGVGSSSGNWHCDSQWLGDRVITTSTRTWALPTYNNHLYKQISNSTSGGSSNDNAYFGYSTPWGYFDFNRFHCHFSPRDWQRLINNNWGFRPKRLNFKLFNIQVKEVTDNNGVKTIANNLTSTVQVFTDSDYQLPYVLGSAHEGCLPPFPADVFMIPQYGYLTLNDGSQAVGRSSFYCLEYFPSQMLRTGNNFQFSYEFENVPFHSSYAHSQSLDRLMNPLIDQYLYYLSKTINGSGQNQQTLKFSVAGPSNMAVQGRNYIPGPSYRQQRVSTTVTQNNNSEFAWPGASSWALNGRNSLMNPGPAMASHKEGEDRFFPLSGSLIFGKQGTGRDNVDADKVMITNEEEIKTTNPVATESYGQVATNHQSAQAQAQTGWVQNQGILPGMVWQDRDVYLQGPIWAKIPHTDGNFHPSPLMGGFGMKHPPPQILIKNTPVPADPPTAFNKDKLNSFITQYSTGQVSVEIEWELQKENSKRWNPEIQYTSNYYKSNNVEFAVNTEGVYSEPRPIGTRYLTRNL

SEQ ID NO: 44 - protein, 599 aa, Adeno-associated virus serotype 9
TAPGKKRPVEQSPQEPDSSAGIGKSGAQPAKKRLNFGQTGDTESVPDPQPIGEPPAAPSGVGSLTMASGGGAPVADNNEGADGVGSSSGNWHCDSQWLGDRVITTSTRTWALPTYNNHLYKQISNSTSGGSSNDNAYFGYSTPWGYFDFNRFHCHFSPRDWQRLINNNWGFRPKRLNFKLFNIQVKEVTDNNGVKTIANNLTSTVQVFTDSDYQLPYVLGSAHEGCLPPFPADVFMIPQYGYLTLNDGSQAVGRSSFYCLEYFPSQMLRTGNNFQFSYEFENVPFHSSYAHSQSLDRLMNPLIDQYLYYLSKTINGSGQNQQTLKFSVAGPSNMAVQGRNYIPGPSYRQQRVSTTVTQNNNSEFAWPGASSWALNGRNSLMNPGPAMASHKEGEDRFFPLSGSLIFGKQGTGRDNVDADKVMITNEEEIKTTNPVATESYGQVATNHQSAQAQAQTGWVQNQGILPGMVWQDRDVYLQGPIWAKIPHTDGNFHPSPLMGGFGMKHPPPQILIKNTPVPADPPTAFNKDKLNSFITQYSTGQVSVEIEWELQKENSKRWNPEIQYTSNYYKSNNVEFAVNTEGVYSEPRPIGTRYLTRNL

SEQ ID NO: 45 - protein, 534 aa, Adeno-associated virus serotype 9
MASGGGAPVADNNEGADGVGSSSGNWHCDSQWLGDRVITTSTRTWALPTYNNHLYKQISNSTSGGSSNDNAYFGYSTPWGYFDFNRFHCHFSPRDWQRLINNNWGFRPKRLNFKLFNIQVKEVTDNNGVKTIANNLTSTVQVFTDSDYQLPYVLGSAHEGCLPPFPADVFMIPQYGYLTLNDGSQAVGRSSFYCLEYFPSQMLRTGNNFQFSYEFENVPFHSSYAHSQSLDRLMNPLIDQYLYYLSKTINGSGQNQQTLKFSVAGPSNMAVQGRNYIPGPSYRQQRVSTTVTQNNNSEFAWPGASSWALNGRNSLMNPGPAMASHKEGEDRFFPLSGSLIFGKQGTGRDNVDADKVMITNEEEIKTTNPVATESYGQVATNHQSAQAQAQTGWVQNQGILPGMVWQDRDVYLQGPIWAKIPHTDGNFHPSPLMGGFGMKHPPPQILIKNTPVPADPPTAFNKDKLNSFITQYSTGQVSVEIEWELQKENSKRWNPEIQYTSNYYKSNNVEFAVNTEGVYSEPRPIGTRYLTRNL

SEQ ID NO: 46 - protein, 738 aa, Adeno-associated virus serotype 10
MAADGYLPDWLEDNLSEGIREWWDLKPGAPKPKANQQKQDDGRGLVLPGYKYLGPFNGLDKGEPVNAADAAALEHDKAYDQQLKAGDNPYLRYNHADAEFQERLQEDTSFGGNLGRAVFQAKKRVLEPLGLVEEAAKTAPGKKRPVEPSPQRSPDSSTGIGKKGQQPAKKRLNFGQTGESESVPDPQPIGEPPAGPSGLGSGTMAAGGGAPMADNNEGADGVGSSSGNWHCDSTWLGDRVITTSTRTWALPTYNNHLYKQISNGTSGGSTNDNTYFGYSTPWGYFDFNRFHCHFSPRDWQRLINNNWGFRPKRLSFKLFNIQVKEVTQNEGTKTIANNLTSTIQVFTDSEYQLPYVLGSAHQGCLPPFPADVFMIPQYGYLTLNNGSQAVGRSSFYCLEYFPSQMLRTGNNFEFSYTFEDVPFHSSYAHSQSLDRLMNPLIDQYLYYLSRTQSTGGTQGTQQLLFSQAGPANMSAQAKNWLPGPCYRQQRVSTTLSQNNNSNFAWTGATKYHLNGRDSLVNPGVAMATHKDDEERFFPSSGVLMFGKQGAGRDNVDYSSVMLTSEEEIKTTNPVATEQYGVVADNLQQANTGPIVGNVNSQGALPGMVWQNRDVYLQGPIWAKIPHTDGNFHPSPLMGGFGLKHPPPQILIKNTPVPADPPTTFSQAKLASFITQYSTGQVSVEIEWELQKENSKRWNPEIQYTSNYYKSTNVDFAVNTEGTYSEPRPIGTRYLTRNL

SEQ ID NO: 47 - protein, 601 aa, Adeno-associated virus serotype 10
TAPGKKRPVEPSPQRSPDSSTGIGKKGQQPAKKRLNFGQTGESESVPDPQPIGEPPAGPSGLGSGTMAAGGGAPMADNNEGADGVGSSSGNWHCDSTWLGDRVITTSTRTWALPTYNNHLYKQISNGTSGGSTNDNTYFGYSTPWGYFDFNRFHCHFSPRDWQRLINNNWGFRPKRLSFKLFNIQVKEVTQNEGTKTIANNLTSTIQVFTDSEYQLPYVLGSAHQGCLPPFPADVFMIPQYGYLTLNNGSQAVGRSSFYCLEYFPSQMLRTGNNFEFSYTFEDVPFHSSYAHSQSLDRLMNPLIDQYLYYLSRTQSTGGTQGTQQLLFSQAGPANMSAQAKNWLPGPCYRQQRVSTTLSQNNNSNFAWTGATKYHLNGRDSLVNPGVAMATHKDDEERFFPSSGVLMFGKQGAGRDNVDYSSVMLTSEEEIKTTNPVATEQYGVVADNLQQANTGPIVGNVNSQGALPGMVWQNRDVYLQGPIWAKIPHTDGNFHPSPLMGGFGLKHPPPQILIKNTPVPADPPTTFSQAKLASFITQYSTGQVSVEIEWELQKENSKRWNPEIQYTSNYYKSTNVDFAVNTEGTYSEPRPIGTRYLTRNL

SEQ ID NO: 48 - protein, 535 aa, Adeno-associated virus serotype 10
MAAGGGAPMADNNEGADGVGSSSGNWHCDSTWLGDRVITTSTRTWALPTYNNHLYKQISNGTSGGSTNDNTYFGYSTPWGYFDFNRFHCHFSPRDWQRLINNNWGFRPKRLSFKLFNIQVKEVTQNEGTKTIANNLTSTIQVFTDSEYQLPYVLGSAHQGCLPPFPADVFMIPQYGYLTLNNGSQAVGRSSFYCLEYFPSQMLRTGNNFEFSYTFEDVPFHSSYAHSQSLDRLMNPLIDQYLYYLSRTQSTGGTQGTQQLLFSQAGPANMSAQAKNWLPGPCYRQQRVSTTLSQNNNSNFAWTGATKYHLNGRDSLVNPGVAMATHKDDEERFFPSSGVLMFGKQGAGRDNVDYSSVMLTSEEEIKTTNPVATEQYGVVADNLQQANTGPIVGNVNSQGALPGMVWQNRDVYLQGPIWAKIPHTDGNFHPSPLMGGFGLKHPPPQILIKNTPVPADPPTTFSQAKLASFITQYSTGQVSVEIEWELQKENSKRWNPEIQYTSNYYKSTNVDFAVNTEGTYSEPRPIGTRYLTRNL

SEQ ID NO: 49 - protein, 733 aa, Adeno-associated virus serotype 11
MAADGYLPDWLEDNLSEGIREWWDLKPGAPKPKANQQKQDDGRGLVLPGYKYLGPFNGLDKGEPVNAADAAALEHDKAYDQQLKAGDNPYLRYNHADAEFQERLQEDTSFGGNLGRAVFQAKKRVLEPLGLVEEGAKTAPGKKRPLESPQEPDSSSGIGKKGKQPARKRLNFEEDTGAGDGPPEGSDTSAMSSDIEMRAAPGGNAVDAGQGSDGVGNASGDWHCDSTWSEGKVTTTSTRTWVLPTYNNHLYLRLGTTSSSNTYNGFSTPWGYFDFNRFHCHFSPRDWQRLINNNWGLRPKAMRVKIFNIQVKEVTTSNGETTVANNLTSTVQIFADSSYELPYVMDAGQEGSLPPFPNDVFMVPQYGYCGIVTGENQNQTDRNAFYCLEYFPSQMLRTGNNFEMAYNFEKVPFHSMYAHSQSLDRLMNPLLDQYLWHLQSTTSGETLNQGNAATTFGKIRSGDFAFYRKNWLPGPCVKQQRFSKTASQNYKIPASGGNALLKYDTHYTLNNRWSNIAPGPPMATAGPSDGDFSNAQLIFPGPSVTGNTTTSANNLLFTSEEEIAATNPRDTDMFGQIADNNQNATTAPITGNVTAMGVLPGMVWQNRDIYYQGPIWAKIPHADGHFHPSPLIGGFGLKHPPPQIFIKNTPVPANPATTFTAARVDSFITQYSTGQVAVQIEWEIEKERSKRWNPEVQFTSNYGNQSSMLWAPDTTGKYTEPRVIGSRYLTNHL

SEQ ID NO: 50 - protein, 596 aa, Adeno-associated virus serotype 11
TAPGKKRPLESPQEPDSSSGIGKKGKQPARKRLNFEEDTGAGDGPPEGSDTSAMSSDIEMRAAPGGNAVDAGQGSDGVGNASGDWHCDSTWSEGKVTTTSTRTWVLPTYNNHLYLRLGTTSSSNTYNGFSTPWGYFDFNRFHCHFSPRDWQRLINNNWGLRPKAMRVKIFNIQVKEVTTSNGETTVANNLTSTVQIFADSSYELPYVMDAGQEGSLPPFPNDVFMVPQYGYCGIVTGENQNQTDRNAFYCLEYFPSQMLRTGNNFEMAYNFEKVPFHSMYAHSQSLDRLMNPLLDQYLWHLQSTTSGETLNQGNAATTFGKIRSGDFAFYRKNWLPGPCVKQQRFSKTASQNYKIPASGGNALLKYDTHYTLNNRWSNIAPGPPMATAGPSDGDFSNAQLIFPGPSVTGNTTTSANNLLFTSEEEIAATNPRDTDMFGQIADNNQNATTAPITGNVTAMGVLPGMVWQNRDIYYQGPIWAKIPHADGHFHPSPLIGGFGLKHPPPQIFIKNTPVPANPATTFTAARVDSFITQYSTGQVAVQIEWEIEKERSKRWNPEVQFTSNYGNQSSMLWAPDTTGKYTEPRVIGSRYLTNHL

SEQ ID NO: 51 - protein, 537 aa, Adeno-associated virus serotype 11
MRAAPGGNAVDAGQGSDGVGNASGDWHCDSTWSEGKVTTTSTRTWVLPTYNNHLYLRLGTTSSSNTYNGFSTPWGYFDFNRFHCHFSPRDWQRLINNNWGLRPKAMRVKIFNIQVKEVTTSNGETTVANNLTSTVQIFADSSYELPYVMDAGQEGSLPPFPNDVFMVPQYGYCGIVTGENQNQTDRNAFYCLEYFPSQMLRTGNNFEMAYNFEKVPFHSMYAHSQSLDRLMNPLLDQYLWHLQSTTSGETLNQGNAATTFGKIRSGDFAFYRKNWLPGPCVKQQRFSKTASQNYKIPASGGNALLKYDTHYTLNNRWSNIAPGPPMATAGPSDGDFSNAQLIFPGPSVTGNTTTSANNLLFTSEEEIAATNPRDTDMFGQIADNNQNATTAPITGNVTAMGVLPGMVWQNRDIYYQGPIWAKIPHADGHFHPSPLIGGFGLKHPPPQIFIKNTPVPANPATTFTAARVDSFITQYSTGQVAVQIEWEIEKERSKRWNPEVQFTSNYGNQSSMLWAPDTTGKYTEPRVIGSRYLTNHL

SEQ ID NO: 52 - protein, 742 aa, Adeno-associated virus serotype 12
MAADGYLPDWLEDNLSEGIREWWALKPGAPQPKANQQHQDNGRGLVLPGYKYLGPFNGLDKGEPVNEADAAALEHDKAYDKQLEQGDNPYLKYNHADAEFQQRLATDTSFGGNLGRAVFQAKKRILEPLGLVEEGVKTAPGKKRPLEKTPNRPTNPDSGKAPAKKKQKDGEPADSARRTLDFEDSGAGDGPPEGSSSGEMSHDAEMRAAPGGNAVEAGQGADGVGNASGDWHCDSTWSEGRVTTTSTRTWVLPTYNNHLYLRIGTTANSNTYNGFSTPWGYFDFNRFHCHFSPRDWQRLINNNWGLRPKSMRVKIFNIQVKEVTTSNGETTVANNLTSTVQIFADSTYELPYVMDAGQEGSFPPFPNDVFMVPQYGYCGVVTGKNQNQTDRNAFYCLEYFPSQMLRTGNNFEVSYQFEKVPFHSMYAHSQSLDRMMNPLLDQYLWHLQSTTTGNSLNQGTATTTYGKITTGDFAYYRKNWLPGACIKQQKFSKNANQNYKIPASGGDALLKYDTHTTLNGRWSNMAPGPPMATAGAGDSDFSNSQLIFAGPNPSGNTTTSSNNLLFTSEEEIATTNPRDTDMFGQIADNNQNATTAPHIANLDAMGIVPGMVWQNRDIYYQGPIWAKVPHTDGHFHPSPLMGGFGLKHPPPQIFIKNTPVPANPNTTFSAARINSFLTQYSTGQVAVQIDWEIQKEHSKRWNPEVQFTSNYGTQNSMLWAPDNAGNYHELRAIGSRFLTHHL

SEQ ID NO: 53 - protein, 605 aa, Adeno-associated virus serotype 12
TAPGKKRPLEKTPNRPTNPDSGKAPAKKKQKDGEPADSARRTLDFEDSGAGDGPPEGSSSGEMSHDAEMRAAPGGNAVEAGQGADGVGNASGDWHCDSTWSEGRVTTTSTRTWVLPTYNNHLYLRIGTTANSNTYNGFSTPWGYFDFNRFHCHFSPRDWQRLINNNWGLRPKSMRVKIFNIQVKEVTTSNGETTVANNLTSTVQIFADSTYELPYVMDAGQEGSFPPFPNDVFMVPQYGYCGVVTGKNQNQTDRNAFYCLEYFPSQMLRTGNNFEVSYQFEKVPFHSMYAHSQSLDRMMNPLLDQYLWHLQSTTTGNSLNQGTATTTYGKITTGDFAYYRKNWLPGACIKQQKFSKNANQNYKIPASGGDALLKYDTHTTLNGRWSNMAPGPPMATAGAGDSDFSNSQLIFAGPNPSGNTTTSSNNLLFTSEEEIATTNPRDTDMFGQIADNNQNATTAPHIANLDAMGIVPGMVWQNRDIYYQGPIWAKVPHTDGHFHPSPLMGGFGLKHPPPQIFIKNTPVPANPNTTFSAARINSFLTQYSTGQVAVQIDWEIQKEHSKRWNPEVQFTSNYGTQNSMLWAPDNAGNYHELRAIGSRFLTHHL

SEQ ID NO: 54 - protein, 537 aa, Adeno-associated virus serotype 12
MRAAPGGNAVEAGQGADGVGNASGDWHCDSTWSEGRVTTTSTRTWVLPTYNNHLYLRIGTTANSNTYNGFSTPWGYFDFNRFHCHFSPRDWQRLINNNWGLRPKSMRVKIFNIQVKEVTTSNGETTVANNLTSTVQIFADSTYELPYVMDAGQEGSFPPFPNDVFMVPQYGYCGVVTGKNQNQTDRNAFYCLEYFPSQMLRTGNNFEVSYQFEKVPFHSMYAHSQSLDRMMNPLLDQYLWHLQSTTTGNSLNQGTATTTYGKITTGDFAYYRKNWLPGACIKQQKFSKNANQNYKIPASGGDALLKYDTHTTLNGRWSNMAPGPPMATAGAGDSDFSNSQLIFAGPNPSGNTTTSSNNLLFTSEEEIATTNPRDTDMFGQIADNNQNATTAPHIANLDAMGIVPGMVWQNRDIYYQGPIWAKVPHTDGHFHPSPLMGGFGLKHPPPQIFIKNTPVPANPNTTFSAARINSFLTQYSTGQVAVQIDWEIQKEHSKRWNPEVQFTSNYGTQNSMLWAPDNAGNYHELRAIGSRFLTHHL

SEQ ID NO: 55 - protein, 738 aa, Adeno-associated virus serotype rh10
MAADGYLPDWLEDNLSEGIREWWDLKPGAPKPKANQQKQDDGRGLVLPGYKYLGPFNGLDKGEPVNAADAAALEHDKAYDQQLKAGDNPYLRYNHADAEFQERLQEDTSFGGNLGRAVFQAKKRVLEPLGLVEEGAKTAPGKKRPVEPSPQRSPDSSTGIGKKGQQPAKKRLNFGQTGDSESVPDPQPIGEPPAGPSGLGSGTMAAGGGAPMADNNEGADGVGSSSGNWHCDSTWLGDRVITTSTRTWALPTYNNHLYKQISNGTSGGSTNDNTYFGYSTPWGYFDFNRFHCHFSPRDWQRLINNNWGFRPKRLNFKLFNIQVKEVTQNEGTKTIANNLTSTIQVFTDSEYQLPYVLGSAHQGCLPPFPADVFMIPQYGYLTLNNGSQAVGRSSFYCLEYFPSQMLRTGNNFEFSYQFEDVPFHSSYAHSQSLDRLMNPLIDQYLYYLSRTQSTGGTAGTQQLLFSQAGPNNMSAQAKNWLPGPCYRQQRVSTTLSQNNNSNFAWTGATKYHLNGRDSLVNPGVAMATHKDDEERFFPSSGVLMFGKQGAGKDNVDYSSVMLTSEEEIKTTNPVATEQYGVVADNLQQQNAAPIVGAVNSQGALPGMVWQNRDVYLQGPIWAKIPHTDGNFHPSPLMGGFGLKHPPPQILIKNTPVPADPPTTFSQAKLASFITQYSTGQVSVEIEWELQKENSKRWNPEIQYTSNYYKSTNVDFAVNTDGTYSEPRPIGTRYLTRNL

SEQ ID NO: 56 - protein, 601 aa, Adeno-associated virus serotype rh10
TAPGKKRPVEPSPQRSPDSSTGIGKKGQQPAKKRLNFGQTGDSESVPDPQPIGEPPAGPSGLGSGTMAAGGGAPMADNNEGADGVGSSSGNWHCDSTWLGDRVITTSTRTWALPTYNNHLYKQISNGTSGGSTNDNTYFGYSTPWGYFDFNRFHCHFSPRDWQRLINNNWGFRPKRLNFKLFNIQVKEVTQNEGTKTIANNLTSTIQVFTDSEYQLPYVLGSAHQGCLPPFPADVFMIPQYGYLTLNNGSQAVGRSSFYCLEYFPSQMLRTGNNFEFSYQFEDVPFHSSYAHSQSLDRLMNPLIDQYLYYLSRTQSTGGTAGTQQLLFSQAGPNNMSAQAKNWLPGPCYRQQRVSTTLSQNNNSNFAWTGATKYHLNGRDSLVNPGVAMATHKDDEERFFPSSGVLMFGKQGAGKDNVDYSSVMLTSEEEIKTTNPVATEQYGVVADNLQQQNAAPIVGAVNSQGALPGMVWQNRDVYLQGPIWAKIPHTDGNFHPSPLMGGFGLKHPPPQILIKNTPVPADPPTTFSQAKLASFITQYSTGQVSVEIEWELQKENSKRWNPEIQYTSNYYKSTNVDFAVNTDGTYSEPRPIGTRYLTRNL

SEQ ID NO: 57 - protein, 535 aa, Adeno-associated virus serotype rh10
MAAGGGAPMADNNEGADGVGSSSGNWHCDSTWLGDRVITTSTRTWALPTYNNHLYKQISNGTSGGSTNDNTYFGYSTPWGYFDFNRFHCHFSPRDWQRLINNNWGFRPKRLNFKLFNIQVKEVTQNEGTKTIANNLTSTIQVFTDSEYQLPYVLGSAHQGCLPPFPADVFMIPQYGYLTLNNGSQAVGRSSFYCLEYFPSQMLRTGNNFEFSYQFEDVPFHSSYAHSQSLDRLMNPLIDQYLYYLSRTQSTGGTAGTQQLLFSQAGPNNMSAQAKNWLPGPCYRQQRVSTTLSQNNNSNFAWTGATKYHLNGRDSLVNPGVAMATHKDDEERFFPSSGVLMFGKQGAGKDNVDYSSVMLTSEEEIKTTNPVATEQYGVVADNLQQQNAAPIVGAVNSQGALPGMVWQNRDVYLQGPIWAKIPHTDGNFHPSPLMGGFGLKHPPPQILIKNTPVPADPPTTFSQAKLASFITQYSTGQVSVEIEWELQKENSKRWNPEIQYTSNYYKSTNVDFAVNTDGTYSEPRPIGTRYLTRNL

SEQ ID NO: 58 - protein, 25 aa, synthetic construct
GGGGSGGGGSGGGGSGGGGSGGGGS

SEQ ID NO: 59 - protein, 5 aa, synthetic construct
GGGGS

SEQ ID NO: 60 - protein, 595 aa, Homo sapiens
MPACCSWNDVLQYETNKVTRIQSTNYGTVKWVLHMIVFSYISFALVSDKLYQRKEPVISSVHTKVKGIAEVTENVTEGGVTKLGHSIFDTADYTFPLQGNSFFVMTNYVKSEGQVQTLCPEYPRRGAQCSSDRRCKKGWMDPQSKGIQTGRCVPYDKTRKTCEVSAWCPTEEEKEAPRPALLRSAENFTVLIKNNIHFPGHNYTTRNILPTMNGSCTFHKTWDPQCSIFRLGDIFQEAGENFTEVAVQGGIMGIEIYWDCNLDSWSHHCRPRYSFRRLDDKNTDESFVPGYNFRYAKYYKENNVEKRTLIKAFGIRFDILVFGTGGKFDIIQLVVYIGSTLSYFGLATVCIDLLINTYSSAFCRSGVYPYCKCCEPCTVNEYYYRKKCESIMEPKPTLKYVSFVDEPHIRMVDQQLLGKSLQVVKGQEVPRPQMDFSDLSRLSLSLHDSPLTPGQSEEIQLLHEEVAPKSGDSPSWCQCGNCLPSRLPEQRRALEELCCRRKPGRCITTSKLFHKLVLSRDTLQLLLLYQDPLLVLGEEATNSRLRHRAYRCYATWRFGSQDMADFAILPSCCRWRIRKEFPKTEGQYSGFKYPY

SEQ ID NO: 61 - protein, 300 aa, Homo sapiens
MANCEFSPVSGDKPCCRLSRRAQLCLGVSILVLILVVVLAVVVPRWRQQWSGPGTTKRFPETVLARCVKYTEIHPEMRHVDCQSVWDAFKGAFISKHPCNITEEDYQPLMKLGTQTVPCNKILLWSRIKDLAHQFTQVQRDMFTLEDTLLGYLADDLTWCGEFNTSKINYQSCPDWRKDCSNNPVSVFWKTVSRRFAEAACDVVHVMLNGSRSKIFDKNSTFGSVEVHNLQPEKVQTLEAWVIHGGREDSRDLCQDPTIKELESIISKRNIQFSCKNIYRPDKFLQCVKNPEDSSCTSEI

SEQ ID NO: 62 - protein, 290 aa, Mus musculus
MRIFAGIIFTACCHLLRAFTITAPKDLYVVEYGSNVTMECRFPVERELDLLALVVYWEKEDEQVIQFVAGEEDLKPQHSNFRGRASLPKDQLLKGNAALQITDVKLQDAGVYCCIISYGGADYKRITLKVNAPYRKINQRISVDPATSEHELICQAEGYPEAEVIWTNSDHQPVSGKRSVTTSRTEGMLLNVTSSLRVNATANDVFYCTFWRSQPGQNHTAELIIPELPATHPPQNRTHWVLLGSILLFLIVVSTVLLFLRKQVRMLDVEKCGVEDTSSKNRNDTQFEET

SEQ ID NO: 63 - protein, 574 aa, Homo sapiens
MCPRAARAPATLLLALGAVLWPAAGAWELTILHTNDVHSRLEQTSEDSSKCVNASRCMGGVARLFTKVQQIRRAEPNVLLLDAGDQYQGTIWFTVYKGAEVAHFMNALRYDAMALGNHEFDNGVEGLIEPLLKEAKFPILSANIKAKGPLASQISGLYLPYKVLPVGDEVVGIVGYTSKETPFLSNPGTNLVFEDEITALQPEVDKLKTLNVNKIIALGHSGFEMDKLIAQKVRGVDVVVGGHSNTFLYTGNPPSKEVPAGKYPFIVTSDDGRKVPVVQAYAFGKYLGYLKIEFDERGNVISSHGNPILLNSSIPEDPSIKADINKWRIKLDNYSTQELGKTIVYLDGSSQSCRFRECNMGNLICDAMINNNLRHTDEMFWNHVSMCILNGGGIRSPIDERNNGTITWENLAAVLPFGGTFDLVQLKGSTLKKAFEHSVHRYGQSTGEFLQVGGIHVVYDLSRKPGDRVVKLDVLCTKCRVPSYDPLKMDEVYKVILPNFLANGGDGFQMIKDELLRHDSGDQDINVVSTYISKMKVIYPAVEGRIKFSTGSHCHGSFSLIFLSLWAVIFVLYQ

SEQ ID NO: 64 - protein, 5 aa, synthetic construct
AAAGA

SEQ ID NO: 65 - protein, 5 aa, synthetic construct
GGGGA